European Patent Specification EP 3 567 107 B1, published June 11, 2025. Title: A gene involved in production of a cyclic peptide, a method for producing the cyclic peptide using the same, and a transformant comprising the same. Applicant: National Institute of Advanced Industrial Science and Technology Tohoku University Kumiai Chemical Industry Co., Ltd. The sequence listing filed with the application follows.

SEQUENCE LISTING (151 sequences)

SEQ ID NO: 1 - protein, 393 aa, Curvularia clavata
LTFAELDSFSSCLAQHIQSLELGDAKAIPLCFEKSKWAIVGMLGVLKAGRAFTLIDPSNPPARARQICRQTAATISIASPYQCDMMRALVPDCIVVDDDFFKSLAFDTDQFQPTATPQTLAYILFTSGSTGEPKGSMMEHHGFVSCCLEFGAALGINSNTRALQFASYAFGACLLEILTTLMHGGTVCIPSDDERINDAPGFIRRANVNWAILTPSFIGAIQPTTVPNLKTLVLVGEAMPSDIRDVWASHVQLKNAYGQSESATICSVTEVTPATVEAHNIGHAVGARFWITDPNNPNKLAPIGCVGELLVESPGIARGYLIPLPADATPFIDTLPDWYPRTQPLDNFKFYRTGDLVCYRSDGTVVYLGRRDSQIKIRGQRVEIGEVETCLRQ

SEQ ID NO: 2 - protein, 69 aa, Curvularia clavata
ITLERIWFQSLGLKPNSTRHKSNFFNLGGDSIAAIRMVNMARAAGLLLSISDIFQNPSLAGLINVMQQS

SEQ ID NO: 3 - protein, 298 aa, Curvularia clavata
GPVEQSFAQGRLWFLDQLTTGASWYLMPLAVRIHGPLRVQALSSALHALEQRHETLRTTFEQQDGMGVQIVHPSSKRELRVIDVSGKQNGGYDQVLKREQTTPIDLAKEPGWRAALLRVGDDEHILSIVIHHIIYDGWSLGVLREELGDLYAAALRGPDPLAHMAPLPIQYRDFSVWQKQPQQVAQHQQQLVYWTKQLEDSAPAELLTDFPRPAELSGRAGEVRFTIEGSVFDSLLAFRRVHQTTSFAVLLAVFRAAHYRLTGTEDATIGTPIANRTRAEVEKLIGFFVNTQCMRIAV

SEQ ID NO: 4 - protein, 398 aa, Curvularia clavata
LTYAQLDQESDKIAVWLRKRNIPAETLIALLAPRSCDSVAAFLGILKANLAYLPLDVNVPAARIEAILSTVAGHKLVLLGRDVPLLGTQLADLELVRIGEALRGSSSGSVAADKAIRPTATSLAYVIFTSGSTGQPKGIMVPHRSLVNVIKQRPAYGNVAHMTNLAFDPSLFEMCTALFNGNTLICIDTLVALDATQLPTIFKQEAIRVAMMTPALLTRLLAQATDALHELEALYVLGDRFPPKDAARASELVKTAVYNAYGPSENSICTTLFHAATGAMCTNGVPVGRVINNSGVYVMDPKQSLVSYGVMGELVVAGEGLAIGYTKPELNEGRFLTLTMDGKPVRAFRTGDRVRYRPTDGQLEFFGRMDFQIKIRGHRVELAEVERVLNRHPAIKDA

SEQ ID NO: 5 - protein, 69 aa, Curvularia clavata
IEAVLCEEFAHILGVEIGVTDNFFDLGGHSLMATTLAARLARRLNASISVKDVFDQPIVANLAATIKRG

SEQ ID NO: 6 - protein, 297 aa, Curvularia clavata
GPVEQSFAQGRLWFLDQLNLGAAWYHMPLAVRLRGPLHLEALTAALHALEERHETLRTVFEEQDGVGMQIVRPSSKTPLRIIDVSTKERGYAELLKQEQTTPFDLATELGWRVALLRQGKDDHILSIVIHHIISDGWSLDILCEELGQFYAAVLRGQDPLAQISPLPIQYRDFSLWQKQPEQVAEHHRQLEYWTTQLEGSVPAELLTDLPRPTIQSGKAGVIPITVNGPVYERLRAFSRAHQTTAFAVLLAAFRATHYRLSGVADATIGTPIANRNRPELENMIGFFVNAQCMRITV

SEQ ID NO: 7 - protein, 402 aa, Curvularia clavata
LTYAQLNEQSDKVAAWLHQCNLPTETLVAVLAPRSCQTVVAFLGILKANLAYLPLDVNVPAARIEAILSEVSGHILVLLGSHVSAPKIELADVEFVKIDNTVEHNLPGRIGSAPSATSLAYVIFTSGSTGKPKGVKVEHRGIVRLVKESNVVAKMPQAARIAHLSNIAFDAATWELYAALLNGGTLVCINYLTTLDSKALEAVFEQEKIQAAMLPPALLKQYLVNIPAAIGALEVVLVAGDRFDRRDAAATQALVGAGVYNAYGPTENTTLSTIYNVVQGDANVNGVPIGRPVSNSGAYIMNMNQELVPIGVIGELVVVGDGVARGYTDPALDVNRFVNVTIEGQTMRAYRTGDRARYRPKDAQIEFFGRMDQQIKIRGHRIEPAEVEHALLNNDLLQDAAV

SEQ ID NO: 8 - protein, 224 aa, Curvularia clavata
DGSAIDKAEMQEWLDDTMQTILDGRPAGRVLEIGTGTGMILFNLGEGLQSYVGLEPSTSAAAFVNRRIQTLPAFAGKAEVHVGTATDISQLQDLRPEVVVINSVAQYFPSPEYLSKVLYALAQIPGVKRLFFGDMRSYAINDQFLAARALHNIGSKATKSAIRSKMVDLENSEEELLVDPTFFTNLATELPEVEHVEILPKRMQATNELSAYRYAAVVHIRDSS

SEQ ID NO: 9 - protein, 69 aa, Curvularia clavata
TEAVLCEEFTDVLGLEVGITDNFFDLGGHSLMATKLAARISRRLDARVSVKDVFDQPVIVDLAASIRRG

SEQ ID NO: 10 - protein, 295 aa, Curvularia clavata
GPVEQSFAQGRLWFLDQLNLGASLYLMPLALRLRGPLRIDALTAALFALEQRHETLRTVFKEQDGVGIQIIQPSQKKKLRTIDVSAGDFSEALHHERTAPFDLASEPGFRVALLQLEPSDHVLSIVMHHIIYDGWSIDILCQELGQFYAAAIQGQDPLGQVSPLPIQYRDFSVWQKQPEQVAEHERQLAYWIDQLADSAPAEFLVDLPRPPVLSGDAGLVHLTIDGPIYDRLRAFCRVHQTTTFAVLLAAFRATHYRLTGAEDATVGTPIANRNRPELENLVGFFVNTQCMRISV

SEQ ID NO: 11 - protein, 404 aa, Curvularia clavata
LTYAQLDEQSDEVAVWLHQRKLPAESLVAVLAPRSCETIITFFGILKANLAYLPLDINVPAARIQAILSSVAGKKILLLGSDQAQPEIRLDDVEFVQINETIDHNMAKDNTTRSGPLATSLAYVIFTSGSTGQPKGVKVEHRGIVRLVKNSNVVAKMPEAACVAHLSNLAFDAATWEIYAALLNGGSLICIDYFTTLDSKVLEAVFEREQIRAAMFPPALLKQCLLNIPTTISALDVILAAGDRFDRRDAIAAQALVGGGVYNAYGPTENTTLSTIYNVVDGDTNVNGIPIGLPVSNSGVYVMDPNQQLVPLGVMGELVVVGDGVARGYTDPALDVDRFIKVEIDGQIVRAYRTGDRVRHRPKDGQIEFFGRMDQQVKIRGHRIELAEVEHVILDNSLVQDAAV

SEQ ID NO: 12 - protein, 69 aa, Curvularia clavata
IETILCEEYAEVLGVEVGVMDNFFDLGGHSLMATKLAARATRRLDAKLSVKDIFDYPILANLAAAVQRG

SEQ ID NO: 13 - protein, 298 aa, Curvularia clavata
GPVEQSFAQGRLWFLDQLNVGSNWYLQPIAIRIRGSLNINALTTALHALEQRHETLRTTFEEEDGVGMQVVQEYDPIELRIMDIAADYDGDYTEALKGEQTTPFDLESEPGWRVSLLRMNDNDHILSLVLHHIISDGWSVDVLRQELKQFYAAALQGLDPLSGADPLPIQYRDFSLWQKQPEQVAEHERQLKYWVEQLADNSPATLLADRPRPSVLSGQAGSVPLSIEGQVYEKLQAFCRAHQTTSFSVLLAAFRAAHFRLTGVDDATIGIPIANRNRPELEHLIGFFVNRQCMRITV

SEQ ID NO: 14 - protein, 403 aa, Curvularia clavata
LTYAQLDQQSDEIATWLRNKKMAPETLVGVLAPRSCQTIVAFLGVLKANLAYLPLDVNAPMARVETIMSSVPGSKLLLLGSDVPAQEIQLQNVELVRIEDTLGHAASAGTATTEPSPTSLAYVIFTSGSTGKPKGVMVEHRSVIRLVRKESNSMSKMSSRARVAHLTNIAFDVSAWEVYATLLNGGTLVCVDYFTSFDAKALGLLFEREQITAAMITPTLLKQCITIVPEALRKLSVLYTGGDRFDRRDAIATKALVKGPVYNAWGPTETTIVSTIYELADDDQFTNGVPIGKAVSNSWAYVMDLNQQLVPVGVMGEAVVIGDGLARGYTDPALDCNRFVHITIDGKRVRAYRTGDRARYRPKDGEIEFFGRMDRQLKIRGHRIEPAEIEHAMLGHNDIVDVA

SEQ ID NO: 15 - protein, 224 aa, Curvularia clavata
DGGAIDQAEMQEWLDDTIQTIVDGQPAGHVFEIGTGTGMIMFGLGKQGLQSYVGLEPSTSATTYVNRKIKTAPTVAGKAKVYVGTAMEAAQLNGLHPEVVVINSVAQYFPTPEYLLEVVGILTQMPGVKRLFFGDIRSYATNRKFLAARALHMLGSNAKKHDIRRKMAELDEFEEELIVDPSFFTGLVSRLPGQVKHVEILPKQMIATNELSAYRYAAVVHLAL

SEQ ID NO: 16 - protein, 69 aa, Curvularia clavata
VEAVLCEEFSEVLGVEVGVTDNFFDLGGHSLMATKLAARTGRRLDAKVSVKDVFDHPVLADLAAAIQRG

SEQ ID NO: 17 - protein, 298 aa, Curvularia clavata
GPVEQSYAQGRLWFLEQLNFKATWYLLPLAVRIRGPLNIKALTTALHALEQRHETLRTTFIERDGVGKQAVQPFQPKELEIVDIAADHQGDYLKVLRDEQTTMFNLATQPGWRVTLHRVDQNTHNLSIVMHHIISDGWSVDVLRHELRQFYAAALRGQDPLAHISPLPIQYRDFSLWQKQPDQIIEHAKQLEYWTKQLADSSPAELPTDLPRPAVLSGKAGEVALSVKGPLYERLQAFCKTHQTTAFATLLAAFRATHHRLTGAEDATIGTPIANRNRPELENLIGFFVNAQCMRITI

SEQ ID NO: 18 - protein, 402 aa, Curvularia clavata; identical to SEQ ID NO: 7

SEQ ID NO: 19 - protein, 222 aa, Curvularia clavata
DGSAIDKAEMQEWLDDTMQTILDGRPAGRVLEIGTGTGMILFNLGEGLQSYVGLEPSTSAAAFVNRRIQTLPAFAGKAEVHVGTATDISQLQDLRPEVVVINSVAQYFPSPEYLSKVLYALAQIPGVKRLFFGDMRSYAINDQFLAARALHNIGSKATKSAIRSKMVDLENSEEELLVDPTFFTNLATELPEVEHVEILPKRMQATNELSAYRYAAVVHIRD

SEQ ID NO: 20 - protein, 69 aa, Curvularia clavata
IEAALCEVFVDLLGTEVSITDNFFNLGGHSLMATKLAARISRRLDARISVKDVFDYPVLADLAGAVQRG

SEQ ID NO: 21 - protein, 295 aa, Curvularia clavata
GPVEQSFAQGRLWFLDQLNAGSLWYIQPIAVRVRGSLNIGALTTALNALEKRHEPLRTTFEEHDGIGVQVVQPHQPKKLRIVDTVANYQGDFIRALRKEQQTLFNLATEPGWRVSLLRIGEDDNILSIVMHHIISDGWSVDILRQDLKLFYAAALKSQEPQVDALPIQYRDFAFWQKQPEQVAEHQRQLDYWIEQLKDSKPAELITDFPRPEVLSGTAGIVQLAVDGQVYEGLRAFCRIHQTTSFVVLLAAFRAAHYRLTGTEDATIGSPIANRNRPELESLIGFFVNTQCMRIM

SEQ ID NO: 22 - protein, 406 aa, Curvularia clavata
LTYAQLDEESNKVATWLSQRQLAPETLVGVLAPRSCPTIVTFFGILKASLAYLPLDVNVPSARIEAILSAVPDHKLVFLGADVPDPEAPLVNVELVRIDDILRQSIHASNAGLLANHPLATSLAYVMFTSGSTGKPKGVMVEHRSIVRLVKETNLVPAVEAVSSVAHISNVAFDAATWEIYAALLNGGTTVCIDHITVLDPAKLALVFSSEKIKAAFFSTALLKQRLYEEPSTITGLDLLYAGGERMRPQDALKTRELVRGSFCHVYGPTENTTFSTVYPMGVEERCVNGLPIGRAVSHSGAVIMDANQRLVPLGVMGELVVTGDGLARGYTDPALNRDRFVEVNIHGQVLRAYRTGDQARYRPKDGQIEFSGRMDRQLKIRGHRIEPAEVEHAILSHDDIRNAVV

SEQ ID NO: 23 - protein, 221 aa, Curvularia clavata
DGTAIDKAEMQEWLDDTMRTLHDGRDPGHVLEVGTGTGMILFNLGKGLQSYVGLEPSTSAAAFVNRKIETISSLAGKAKVEIGTATDVGQLKNLRSDLVVINSVAQYFPSPEYLVEAVTALVHIPGVKRLFFGDMRSYAMNKQFLVARALRTLGAKANKDDVRRKMVELEEFEEELLVDPAFFTGLANWLSEVEHVEILPKQMTSTNELSSYRYAAIVHLR

SEQ ID NO: 24 - protein, 69 aa, Curvularia clavata
IEALLCEEFAEVLGVEVGINDDFFDLGGHSLMATKLAARSSRRFDAKVSVKDVFDHPILADLAASIQRG

SEQ ID NO: 25 - protein, 298 aa, Curvularia clavata
GPVEQSFAQGRLWFLEQLNVSSTWYLQPIAVRMRGPLKIEALAAAFHALEERHETLRTTFEEHDGIGMQVVQPHRPKELRVIDVQAEHDGDYTQALHTEQTTTFNLETEPGWRVSVFRLNEDDNILSIVMHHIISDGWSFDILRKEIREFYNAALKGKDPLAQMSPLHIQYRDFSVWQKQLNQITEHKRQLDYWTKNLADNTPAELPTDLPRPAVLSGKAGVIQLSITGPVYDRLRAFCRVHQTTLFTVLLTVFRATHYRLTGAEDATIGTPIANRNRPELENLIGFFVNTQCMRITV

SEQ ID NO: 26 - protein, 405 aa, Curvularia clavata
LTYAQLDLHSDELASWLRQKKMAPETLVGVLAPRSCQTIVTFLGILKASLAYLPLDVKVPVARIEAILSSISGQKLILLGQDVPVPEIQLPDVDVVPISEILGRSVPSRATDKSLGPLARNLAYVLFTSGSTGKPKGVMIEHRSIVRLVKETNLISKLPNAPRTAHLTNLVFDNSAWEIYSTLLNGGTLVCIDYATVLDSKALETVFKEQRIQTSLMPPALLKECLANMPTMFDDVEVLYALGDRFDKQDAMKARSIVKTAVYNAYGPTENTVISTIYEIAKDDSFVNGVPIGRSISNSGAFIMDSRQQLVPVGVLGELVVSGDGLARGYTDPTLDVNRFVEVTVDGQHVRVYRTGDRVRFRPKDGQIEFFSRMDQQVKIRGHRIEPAEVEHVILTNKIIRDAAV

SEQ ID NO: 27 - protein, 69 aa, Curvularia clavata
MERILCEEFADVLGVEVGITDNFFDFGGHSLMATKLAARISRRVNARVSVKSVFDHPVLVDLASTIKQD

SEQ ID NO: 28 - protein, 299 aa, Curvularia clavata
GPVEQSFAQGRLWFLDQLNFGASWYLMPLALRLQGSLHVKSLTTALFALEQRHETLRTTFEEQDGVGIQIVHPANKKDLRILDVSKEQNSDYAKVLHKERTIPIDLTSEPGWRVSLIRLGEDDHILSIVMHHIISDGWSVDVLRQELKQFYTAALKGQDPLAQIDALPIQYRDFSLWQKLPDQVAEHQRQLEYWAEQLADNTPAELLTDLPRPDVLSGKAGAVQLTIDGPVFDQLQAFCRAHQTTMFTVLLAVFRTTHYRLTGATDATIGTPIANRNRPELERLVGFFVNTQCIRITVD

SEQ ID NO: 29 - protein, 403 aa, Curvularia clavata
LTYSQLDDQSDKITAWLLQRKIPAESLVAVYAPRTCQTIITFFGILKANLAYLPLDINVPAARIEAILSTISGHKLVLLGSQVSAPAVQLKDVEYVWIDEAMAETVRTCTSPEPSATSLAYVIFTSGSTGLPKGVKVEHRGVVRLVKQSNVVAKMPQAARVAHLSNIAFDAATWEIYAALLNGGSLICIDYFTTLDSKELEAVFAREKIQAAMLPPALLKQCLVNIPATISALDVVLAAGDRFDRRDAAATQALVGGCVYNAYGPTENTTLSTIYNVVKGDANVNGVPIGRPVSNSGAYIMDPNQQLVPKGVMGELIVVGDGVARGYTDPALDVNRFIEIAIDGDQAVRAYRTGDRARYRPKDGQIEFFGRMDQQIKIRGHRIEPAEVEHAVLDNSMVQDAAV

SEQ ID NO: 30 - protein, 225 aa, Curvularia clavata
DGSAIDKDEMQEWLDDTMSTLLDGRQPGHVLEIGTGTGMILFNLAERMGLKSYVGLDPSEKATSFVKQAIKSRPSLAGKAEVHVGTATDVARMRDLHPEVVVINSVAQYFPSPEYLADVVGALVRIPGVKRLFFGDIRSYATNNHFLAARALHKLGEKATRDTVRSKMAELEGYEEELLVDPTFFTSLTAKLHGQVEHVEILPKRMQATNELSAYRYAAIVYIRD

SEQ ID NO: 31 - protein, 69 aa, Curvularia clavata
VEAVLCEEFTDVLGVEVGITDNFFDLGGHSLMATKLAARISKHLDARVSVKDVFDYPVVADLAASIERN

SEQ ID NO: 32 - protein, 296 aa, Curvularia clavata
GPVEQSFAQGRLWFLDQLNMGVSELYLMPLALRLRGPLRVDAFAAAVSALEARHETLRTTFMDHDGVGMQVILPSNSKKLRVIDASENDYIDILRQERTAPFNLTTEPGFRIALLQLGQTDFILSIVMHHIIYDGWSIDVLCRELGRFYSAALQGQDPLAQVSPLPIQYRDFSIWQKRPEQVAEHERQLQYWTEQLADSSPAELLTDLPRPLVPTGKAGIVQLTIEGAVYERLRAFCRVHQTTSFAVLLAAFRATHYRLTGAEDATIGSPIANRNRPELESLIGFFVNTQCIRVTI

SEQ ID NO: 33 - protein, 405 aa, Curvularia clavata
LTYAQLDEKSDQLAAWLCQHNIPAETIVGVLAPRSCETIIAFLGILKANLAYLPLDDNVPAARIETILSAVPGHTLVLLGSHVAAPSIGLADAEFVNINHTLGHSLQLNSTCAKLQPSATSLAYVIFTSGSTGKPKGVMIEHRSIVRLVKNSNTLAKLPRAARVAHQFNLAFDAANYEIYGTLLNGGALICVDYSTLLDIDALVAMFKREKITASSLSPGLLKQCVNSAPEMLKALQVIYTGGDRLDGRDAIELQALVPGGVYNMYGPTENTVISTLYNLGDKHSYVNGVPIGTTVSNSGAYVMDALQQLVPVGVMGELVVTGDGLARGYTDPELDRNRFIKVNIDGQVVRAYRTGDRVRYRRIDGQLEFFGRMDQQIKIRGFRIETAEVENAMLSHSAVRNAAV

SEQ ID NO: 34 - protein, 67 aa, Curvularia clavata
LEASLCKEFAEVLGVEVGITDNFFDLGGHSLLATKLAARISRRLDTRVSVKDVFDQPVPADLALKVS

SEQ ID NO: 35 - protein, 277 aa, Curvularia clavata
VDVYPVTWIQKHFLVDPATGLPRTPSLFFVDFPANADCDKICNASRSLIQLFDIFRTVFVQAAGNFYQVVLEELDIPISVIETEDISTATRVLKEQDQQNPLQFGQGFLRFAVVKTRSAVRLVLRISHCLYDGLSFEHVVQSLHALYNGDRIPTQPKFVQYVQHLTDSRKEGYDFWLSVLEESSMTVVETGRRAQQLSSPEGAWFVEKIIKAVIPANSDGITQATVFTTASTILLARMTGSSDITFSRLVSGRQSLPINDQHIVGPCTNIVPVRIRM

SEQ ID NO: 36 - DNA, 39126 bp, Curvularia clavata
  CDS (1)..(39126)
atggccagcgacatcaatactcatccagagggagcgaccaagttttggcagcaacactttgacggcttgaacgcctctgtgtttcctgctctgtcctcccatttgactgtcccgcgtcccaacgcgcagacagcacatcgcatttcctattcaaccttggcgaagcaaaaatgggacaacaccagcctttgccgagctgcgctcgcaatactgcttgcccgctattcgaatgcatctgaagcactcttcggcgtcttggtagaacagtttctcccgtccaacggtgaacaggcatcgacagaggaatcaccacaaagcatccttcccatccgcatccgacttgaccttgaggaagctgggttgggccttttgcaagctatcaataccctagatgcatctctgcgcgagtggaagcatatcggtcttgacgccattcgtggcacgggagagtacgggtctgccggatgcgagttccagacagtacttgctgtcactactggaaagacgccacgaacgcatagactcgcgtcttgcactgatcgcgcccttttgctcgattgccgaatggacgacgattcggccacacttctcgcacgctatgatcccagtgtgattgatgacctccaggtcgcccgtttcctaaaacagctcgggcacgtgattgagcaattgcgtgtccaggcagtcgatctacctctctgggaacttggtattgtcacgcaagaagatagcgcagagattcaaaaatggaactcgcagcaactccaattcagccaggaatgcatacacgacgtgttcgccaacagggtggttgatacgccgcagaaaatcgccgtatccgcttggaacggcgagctaacgtttgctgaacttgacagcttctcctcatgcctcgcccagcacatccaatcgcttgaattgggcgatgcaaaagcgataccgctttgctttgagaagtcaaaatgggctatcgtcgggatgctcggtgtgctcaaggctggccgagcattcacactgattgacccatctaacccacccgctagggctcgtcaaatctgtcgacaaacagccgccaccatttccatcgcgtctccataccagtgcgatatgatgcgcgctctggtgcccgactgcatcgtggtcgacgacgactttttcaagtcattggcgtttgatacagatcaattccagcctacggcaacgccgcagacattggcctacatcctcttcacttctggtagtaccggagagccaaaaggcagtatgatggagcatcacggatttgtgtcttgctgtctcgaatttggtgcggcgctgggcatcaacagcaacacacgcgctcttcaatttgcctcttatgctttcggtgcttgcctgctagagattttgaccaccctaatgcacggcggcacggtctgcatcccatctgatgatgaacgcataaatgatgcacccgggtttatcagacgcgcaaacgttaactgggcaattctcactccttctttcattggcgccatccagcccaccaccgtacctaacctcaagacgctggtattggtgggagaagccatgccgtcagacatacgcgatgtctgggcctcgcacgttcagcttaaaaatgcctatggccagagcgagagcgcaacgatctgtagcgtaacggaagtcactcccgcgacggtggaggcgcacaatatcggtcacgctgtgggcgcccgattctggattaccgaccccaataatcccaacaaacttgcgccaatcggctgcgtaggcgagctgcttgttgaaagtcctggcatcgcgcgtggatatctgattcctctgccagcggacgcaacacctttcattgacacgcttcctgattggtacccaaggacgcagccgctcgacaacttcaagttctacagaactggcgatcttgtctgctaccgatccgacggcaccgtggtgtatctggggcgacgagactcgcaaattaagatccgaggacagcgcgtcgaaatcggcgaagtagaaacatgcttgcgacaacagcttcccagtcaactggtaccagttgtcgaagctgtcagtctgtcgggcatgtccaagagcatgacgctgattgcctttctggttggcgaaaacaccattctggaagaggacgtttacgttttggagggcagtgccgcgcagcgcatcagttcgaaactgcgacagattgtacccgggtactgcattccgtctcactatattcgcatcaaccatcttcccactaccgccactggaaagtgtgatcggaaagcacttcgagccatcggtaccaaattgcttagggaagccgtggagggcatggcgtcacaggaggaacaggagagtgcttcgttaatgaccgaagggattacactggaacgcatctggttccagagcctgggtctcaagcccaactccacgagacacaaatctaacttcttcaatctgggcggcgactccattgcggcaatccggatggtgaacatggcacgggcagcaggcttgttgctgagcatctccgatatctttcagaacccctcactggcggggctcatcaatgtgatgcagcagagctcgactgcacaagacgctattcccgccaccgagtacagcgggccggtcgagcagtcgtttgcacagggccgtttgtggttcttggatcagctcacgaccggcgcatcgtggtacctaatgccacttgcggtccgcattcacgggccgctccgcgtccaagccctttccagcgccctgcatgctttggagcagcgccacgagacgctacgaacgacgttcgagcagcaagacggtatgggcgtgcagattgtccacccaagcagcaagagggagctgcgcgtcatcgacgtgtcgggtaagcagaacggcggctacgatcaggtgttgaagcgagagcagacaacacccatcgacttggccaaagagcccggatggagagccgcgctgctacgagtgggcgacgatgagcacatcctctcgattgtcatccaccacatcatatacgacggttggtcgctgggcgtactgcgtgaggaactcggcgacctttatgcggcggcgctgcgaggtcccgatccactcgcacacatggccccgctcccgatccagtaccgcgacttctctgtttggcagaagcagccacagcaagtggcgcagcaccaacaacagctcgtgtactggacaaagcagcttgaagacagcgcgcctgcagagctgcttaccgacttcccccgccctgccgagttatctggccgtgccggtgaggttcgtttcactatcgaaggcagtgtcttcgacagcctgctcgcttttcgtcgcgtccaccagacgacatcatttgcggtgctactagccgtcttccgtgctgcccactatcgtctcaccggcacagaggacgccacaatcggcacgcccatcgctaatcgtactcgtgctgaggtcgagaagctcatcggtttctttgtcaacacgcagtgtatgcgcattgctgtcgccgacgatgacaccttcgcatcgctcgtcagtcaagtctggtccgtcgcgactgccgcattcgagcatcaggatgtccccttcgagcgtatcgtgtcggcgctcctgcccggcgccagagacacatctcgcaacccgctggcccagctcctgtttgcgctccatctggagcaggacctcgacaagatcaatctcgagggcttggcctgcgagactgtacccacgccaatggcgactcgcttcgacgtcgagttccatctcttccaggaagacgacagactgaacggcgtcgtcaacttctccacggacctcttcgagccccagaccatccacagcctggtctctgtctttcaggagatcctgcgccgcggcctcgaccaaccacagacgcctattgcacatctccagctgactgatgggcttgaagagcttcgcaatgccggcctgctggacatcaagaggatcgactacccgcgcgaggcgagcgttgtagacatgttccaaaagcaggtagccgcttgccctaacgtgactgccgtcaaagattcgacctcgcagctcacgtatgctcaactggatcaggagtctgacaagatagccgtttggctgcgcaaacgcaacattccagccgagacattgattgcgctgctagcacctcgatcctgtgactccgtggctgccttcctcggtattctcaaagccaatctggcctatctccctctggatgttaatgtccccgctgctcgtatcgaggcaatcctgtcaaccgtagcaggtcacaaactggtcttgctcggacgagatgtgcctctgctaggtacgcagctggccgacctcgagcttgtccgtatcggcgaggcgctgcgtggctcgagttcagggagtgtcgccgccgacaaggctattcgacctacagcaacaagcctggcctacgttatcttcacgtctggatctactggccagccaaagggtatcatggttcctcatcgcagcttggtcaacgtgatcaagcagcgacctgcctatggaaatgtcgctcacatgacaaatctcgcctttgatccctccctgttcgagatgtgcactgccttgttcaatggcaatacgctgatttgcatcgacacattggtagcactcgatgcaactcagcttcctaccatcttcaagcaggaagcaattcgtgtcgcaatgatgacgccggccttgctcaccagactcctagcccaggctactgacgcactgcatgaactagaggcactttatgttctgggagatcgattccctccaaaagatgctgccagagcaagtgaacttgtcaaaacggccgtatacaatgcctacggaccgagtgagaactccatctgcacaactctcttccatgctgccactggcgccatgtgtaccaatggtgtgcctgttggccgagtaatcaacaactcgggcgtatatgttatggatccaaagcagtcgcttgtttcctacggcgtcatgggtgagctcgtcgtcgctggcgaaggccttgcaattggatataccaagccagaactcaacgaaggccgctttctgacgcttacaatggacggaaaacctgtaagagcgtttcgtaccggagatcgtgttcgataccggccgacagatggtcaactggaattttttggccgcatggacttccaaattaagatccgaggtcatcgtgtcgagttggctgaagtggaacgagttttgaacaggcaccctgccatcaaagacgccatcacactgctgaggcagcacggctcctcagcacaagacacagagcttgtcagttttattgtgctaggagagcagaagcctgtaaagccccatcgaaacgccaccgaccatggcggaatggagattgagcaattggaccaaaagctagaagcaaacctgcgtgccatgatgcaggctacgctgccctcatacatggttccctcgagaatcatagtgctagaccatatgccgctcgacaagaatggaaaggttgaccgacgaggattgacaggactgacgctgagcccagccatggaaacaagctcgcgtgttgttgtggcagcacggaacgagatcgaggccgtactgtgcgaggagtttgctcacatccttggtgttgaaattggcgtcactgataacttcttcgacctcggcggacattcactcatggctactactctcgctgctcgcctcgctcgccgtcttaatgctagcatttccgtcaaggatgtcttcgatcagcctattgtcgctaatctcgccgccacaatcaagcgaggctcgacccctcacaatgcaatccctccaactaaatactctgggccggttgaacagtccttcgcacaaggtcgtctctggtttctggaccaactgaaccttggggctgcctggtatcatatgcctcttgcagtgcgtttgcgcgggcctctccatcttgaggcactcactgcagcgctgcatgcccttgaggagcgccacgagacgttacggacagtatttgaggaacaagatggtgtgggcatgcagatcgtccggccaagcagcaagacgccgctgcgaataatcgacgtgtccactaaagagcgaggttatgccgagttgctcaagcaggagcaaacaacaccattcgatctagccacagagttagggtggagggtggctctgctgaggcaagggaaggatgaccatattctgtcaattgtcattcaccacatcatttccgacggttggtctctcgatatcttgtgcgaggaacttggtcagttctacgccgctgtgctccgtggccaggacccattagcccaaataagccctctgcctatccagtatcgcgatttctctctgtggcagaagcagcctgagcaagttgctgagcaccaccggcaactcgagtactggaccacccagctcgagggcagcgtacctgcagagcttctaaccgatcttcctcgaccaaccatacagtccggcaaggcaggcgtcatcccaataaccgtcaacggccctgtatacgagcgtctacgggccttctctcgagctcatcaaacgaccgcttttgcggtactgttggccgcctttcgagcaactcattaccgtctctctggagtcgcagacgctaccatcggcacgccaatcgccaaccgtaatcgacctgaactggagaatatgataggctttttcgtaaatgcccagtgtatgcgtatcactgtcgagcaagacgatacttttgagacacttgtccgccagatccgatttacggcaactgccgcctttgccaaccaagatgtaccctttgagcatatcgtctcagcccttatgcctgactcacgcgatacatcgcggaatccgctagtgcagctcatgttcgcactccacgcgtacaaagatctcggcaagattgagcttgaaggttatgttgcagagcctgtgcatacaactctgtcaacccgcttcgatctcgaattccacatgttccaggagacaaatcacctcagcggctacgtactgtatgcaacagacttgttcgagcctgagagcattgaggggatggtttccatttttaaagaaatcctcgctcgagctcttgaccaaccccaaaccccactggcgcttctaccgctcaccgatgggctggctgaacttcgcaggagggggctgcttgagattgaaaggcccagctatcctcgcgagtcgagcgttgttgacgtcttctgtagccaggtagcggcttctcccaacgcaaccgctgtgaaggactcgatttcacagctcacttacgctcagctaaatgagcaatctgacaaggtcgctgcttggctacaccagtgcaaccttccaactgaaactttggtcgctgtgctagcgcctcgatcttgccaaacagttgtggccttcttgggtattctgaaggccaacctagcatatcttcccctagacgtcaatgttccggcagctcgcattgaggcaattctctcagaagtctctggccacatacttgtcttacttggatctcatgtttctgctcccaagattgagctcgctgatgtcgaattcgtcaaaattgacaacacagtcgagcacaatttgccgggccgcattggatctgctccatctgccacgagcctcgcctatgttattttcacatctggatcgactggcaagcccaaaggtgttaaggtagagcaccgcggtattgtccgcctcgttaaagagagcaatgtagtagcaaaaatgccacaagctgcgcgcattgctcacttgtcaaacattgcctttgacgcggctacgtgggaattatatgctgcgttgctcaacggcggcaccctcgtctgtatcaactatttaaccacgctggatagtaaagcactcgaggccgtgtttgagcaggaaaagatccaagcggctatgcttccaccagcactgctcaaacagtatttggttaacattcccgcagctatcggtgcactagaagtggtccttgtcgctggtgaccgtttcgatcgacgcgatgctgcagccacgcaggctcttgttggagcaggcgtgtataacgcctatggaccgacggagaatacaacactcagcactatctacaatgtcgttcagggcgatgccaatgtgaatggcgtcccgattggacgccctgtcagcaactctggcgcctacatcatgaatatgaatcaggaactcgttcctattggcgtcataggcgagctggtcgtagtaggagacggtgtcgcccgaggatacaccgacccagccttggacgtcaaccgcttcgtcaacgtcactattgaaggccaaactatgagggcttataggactggcgatcgtgcccgctataggcccaaagacgcacagattgaattctttggccgaatggatcaacagatcaagattcgaggccatcgtattgagccagctgaggtcgagcatgcgttgctcaacaatgacttgcttcaggacgctgcagtcattatccgaaagcaacaaaatgatgagctggagatggttgcttttgtagaagcaaacagcaataagtcgatcgaacaagaggcgagcaaccaagtagaagactggggcgctcaattcgagagcaacgtctacgccgagatcgaggcaatcgatgcctctgctgttggtaacgacttcatgggttggacttccatgtacgacggcagcgcgatcgacaaggctgagatgcaggaatggctcgatgatactatgcagacaatacttgatggtcgaccagccggccgcgttctcgaaatcggcactggcacgggtatgatcctcttcaatcttggtgaagggttacagagctatgtcggtctcgaaccatctacctcggcggctgcgttcgtcaatcgcaggattcagacacttccagctttcgctggtaaagctgaagttcacgtgggtacagcgacagatataagccaacttcaagatctccgcccggaagtagtggttatcaactcggtggctcagtacttcccatcgcctgagtacttgtctaaggttttgtacgcactagcccaaattcctggcgtcaagcgtttgttctttggagacatgcgatcttacgccatcaacgaccagttccttgcagctcgcgccttacacaacataggtagcaaggctactaagagcgccattcgaagcaagatggtcgatctggaaaactctgaggaagaattgctcgtcgacccaaccttcttcaccaacctagcgaccgagcttccagaggttgagcatgttgagattctgccaaaacgcatgcaggctaccaacgaacttagcgcctatcgttatgcagctgtggtgcacatccgtgattcatcggaacgagctcagaccgtgcatgccatcaaatcgagcgcatgggtcgacttcagcaaatctcagatggaccgcaaggccctcatcagtcttcttcaaagctcggtaaacaccgaggctgttgctatcggcaatatcccctacagcaagactatcatggcgcgacatgtcgtccaatcgcttgacgaagacaatgcagacaaggacattgcgcaagataaacccgataagcccacctggatctcggcagttcgctccaatgccgaacactgcccatcactatcggctctcgaccttgtacagcttggtgaggaggcaggcttctgtgtggagctcagctgggctcaacagcgatctcatcacggagcaatcgacgcagtctttcatcattaccagcccgctcgagaaggaagccgtgttctgtttcagttcccgaccgatacgtatcgacgccaatccggtccgcttacaaaccgacccttgcagcgaattcagagccggcgaatggaaacacaggttagagaaaagctacgggccgttttgccttcatacatgattccatcgctcatcgtgctggtcgaccaaatgcccctgaaccccaacggcaaagtggataggaaggcgttggaacgacgagcccaggcagtgctacgggtcgaaaaaccaacttccgaacgtgttggtgcccgtaatgagactgaggctgtgctttgtgaggagtttaccgacgttctcggacttgaggttggtattacggataacttcttcgacctcggtgggcactcgcttatggcgaccaaactcgcggcccgtatcagtcgacgccttgacgcccgcgtctctgttaaagatgtctttgatcagcctgtcatagtcgacctcgccgcctccattcgccgtggttcgacccctcacaatcctatcaccccaaccgagtattctggtccggtagagcaatcgtttgctcagggccgtctctggttcttagaccagttgaatctcggtgcatctttatatctcatgcctcttgcgttgcgtttgcgtggacctctccgcatcgatgctctcacagctgcgctcttcgcattggaacagcgacacgagactctccgaaccgtcttcaaggagcaagatggcgtaggcatccaaatcattcaacctagccaaaagaagaaactcagaaccattgatgtatctgcaggcgacttttccgaggcgctgcatcacgaacgcactgccccatttgatctcgcatcagagccgggcttcagagtcgcccttcttcagcttgagccgtctgatcatgtgctgtctatcgtcatgcaccatatcatctacgacggctggtctatcgacattttgtgtcaagaactgggccagttctacgctgctgcaatccagggccaggatccattgggacaagtgagcccgctcccaattcaataccgtgacttctctgtctggcaaaagcaacctgagcaggtcgctgagcatgagcggcagcttgcgtactggatcgatcagttggccgatagtgctcccgctgagttccttgtcgatctcccacgcccacccgtcttgtctggtgatgccggactagtccacctcactatcgatggtcccatctatgaccgcctgagagccttctgtcgagtgcaccagacgacaacttttgcagtgctactagcagctttccgcgcaacgcactatcgtcttacaggtgccgaagatgctactgttggcacaccaatcgccaaccgtaaccggccggagcttgaaaacttggtcggattcttcgtcaatactcagtgtatgagaattagtgtcggagatgatgacacgtttgagcagctagtgcgccaggttcgatctacagcaacggctgcatttgcaaaccaagacgttccttttgaacgcatcgtgtcaacactcctgccgggctctcgcgataccgcccgcaatccactggtacagctcatgtttgctgtccattctctcaaggaccttggcaaaattcagttcgagggtctcgtgggcgagacaattcccacggcttctttcactcgattcgacgtcgagtttcatttgttccaggaagtcggtcgtcttagcggaaatgtgctcttctcgactgatctatttgagccggagactatccagggcatggtctctgtgttcatggagatcttgcgcggagctcttgaccagcctcagatccccattgccgtcctaccgctcacagacggcctcacggagcttcgcaacagaggcctgcttgaagttgagcagcctcaatatccccgcgactcgagcgtcattgacgtgttccgcgctcaggtcgttgcttgcccagatgcaatcgctgtgaaagattcgacgtcgcagctcacctatgcccaacttgatgagcagtccgatgaggtggctgtatggctacatcaacgaaagttgccagcggaatccctggttgccgtgctagcacctagatcatgcgagactatcattaccttcttcggtattttgaaggctaatctagcctatcttccactcgatattaacgtcccggcagcccgtattcaggcaatcttatcgtccgttgcagggaagaaaatcctcctacttggttctgatcaggctcagccggaaattcggcttgatgatgttgaatttgtacaaatcaatgaaacgattgaccacaatatggcgaaggataatactacccgctctggacccttagctacaagtcttgcttatgttatcttcacttctggatccactggccagccgaagggcgtcaaggtggaacaccgcggtattgttcgcctcgtcaagaatagcaacgtggtagcaaagatgccagaggcggcatgtgttgcacacctttcaaatctcgcgtttgacgccgcgacatgggaaatctacgctgcactcttgaatggtggctcgctcatctgtatcgactacttcaccacgctagacagcaaggtcctcgaggcagttttcgagcgagaacaaatccgtgcagccatgttcccaccggcgcttctgaaacaatgcctactcaatatccccacgaccatcagcgcgctagatgttatcctcgctgctggtgaccgatttgataggcgcgacgctattgcggcgcaggcgcttgttggaggtggtgtatacaatgcctacggtcctacggaaaatactacgcttagcacaatatacaacgttgtggatggcgataccaacgtcaacggtattccaatcgggcttcctgtcagcaactctggcgtgtatgtcatggatcccaaccagcagcttgtcccgttgggcgtcatgggagagcttgttgtggttggcgatggtgtagcccgaggttacactgatccagctcttgatgttgatcgtttcatcaaggttgaaatcgacggccagatcgtacgagcctaccgcactggtgaccgtgttcgacaccgacccaaggacggtcagattgagttctttggccgaatggatcagcaagtcaagattcgaggacatcgcattgaattggctgaggtagagcacgtcatcctcgataacagcttagtccaggacgctgcagtcattgtccacaagcaagctgaccaggagatcgaaatgatcgcatttgctatagtccgaggcgataacgacagcaagcacccagagaaggatattctagatcgagtgaaggctttgcttccatcatacatggtgccagctcaaatggtgctgcttaacagcatgcctctcaatgccaacggcaaggtcgatcgcaaagagcttgctaagagggcggggactgtgccgcgaagcgagatggcatacgtcgctccagagagggttccgcctcgcaatgaaatcgaaacaattctttgcgaagaatacgccgaggtccttggcgtcgaggttggtgtcatggacaactttttcgatcttggagggcactctctcatggcgaccaagcttgcagcccgcgccactcgtcgacttgatgcaaagttgtccgttaaggacatttttgattacccaattttagccaaccttgcagcagcggttcaacgaggctcgactccacataatgcgattctcgcaaccacatactccggaccagttgaacaatcattcgcccaggggcgcctgtggttcttggaccagctgaatgttggctcgaattggtaccttcagccaattgccatacgcatacgcggatcactcaatattaacgcgctcactaccgcgcttcatgccctagaacaacgtcacgagacgttgcgcaccacttttgaggaagaggacggcgttggtatgcaggtcgtccaagaatatgacccgatagagctcaggataatggatattgctgccgattatgacggcgattatacagaagcgttgaagggagagcagacgacccccttcgatctagagtcggagccaggatggagggtatcgctgctccgtatgaacgacaacgatcatatcttgtctctggttctacatcacatcatctccgatggatggtctgtcgacgttctacgccaggagttgaagcaattctatgccgctgcactccaaggcctggatcctctgtcaggggctgatccactccccatccagtaccgcgacttctctctctggcaaaagcagccagagcaagttgctgagcacgaacgacagctcaagtactgggttgagcagttggctgacaattcccctgctacgcttcttgcggaccggccacgtccatctgtgctgtcgggccaagccggctcggtcccgctctctatcgaaggtcaggtctatgagaaacttcaggccttctgccgagctcatcaaacgacctccttttccgttttgctcgctgccttccgagctgctcacttccgcctgacgggtgttgacgacgcgacgattggcataccgatcgccaatcgtaatcgacctgagctagagcacctgatcggctttttcgttaacaggcagtgtatgcggatcacggttggggaagatgatacgttcgaatctcttatccgccaggttcactcaacagccactgcagcgtatgctaatcaagacgtgccgttcgagcgaatcgtatcgtcccttctttctggctcaagagacacatctcgtaatccactcgtccagctagtattcgccgttcactcccagaagaaccttggcaagtttgagttgcaagacttgacatctgagccagttgctggagctatctctactcgatttgatgcggaatttcatctattccaggaagaagagaggttgaacggtgttgtgtattacgcaaccgatctgttcgatgcggagactatccaaggggtggtgtctgttttccaagaaatcttacgtcgcggcctcaaccatccacgaacgccgatcgcagctctgtcgcttacggacgggctggataatcttcgcaagatgaatctggttcacttcaagcggactgattatccccgcgactctagcatggtcgacattttccgcgagcaagtcgctacctatccggacgtgattgctgtcaaggactcgactttacagctgacctacgcgcaacttgatcaacaatccgatgagatagccacctggttgcgaaacaaaaaaatggcgccagaaactctggtgggtgtccttgctccgcgatcgtgccagactatcgtagccttccttggtgtcctcaaggcgaacctagcctatctacctctcgatgtcaatgccccgatggcccgcgttgagacaatcatgtcttctgtgccagggagcaagctgcttcttctaggttctgatgtgcctgcccaggagatccagctgcagaatgttgagttggtgcgtatcgaagacaccctcggccacgctgcctctgccggtacagcgacaacagaaccctctccaaccagcctagcgtacgtcatattcacatctggatcgacgggtaagccaaagggtgtgatggtcgagcatcgaagcgtcattcgcctcgtgagaaaagaaagcaattccatgtccaagatgtcttccagagctcgggttgcgcacttgactaacatcgcgttcgacgtctcagcatgggaggtatatgctacgcttctcaacggagggactctggtctgtgtcgattatttcacttcgttcgatgctaaagccctcggtctgctgttcgagcgggagcagattactgcggctatgatcacgcctacgttgctcaaacagtgcatcactattgtaccagaagctctccgcaagttgtccgttctgtacaccggtggcgatcgctttgataggcgcgatgctatcgcgacaaaagcgcttgtcaagggcccagtttacaatgcatggggccctacagaaaccacaatcgtcagcacaatctatgagcttgccgatgacgatcagttcaccaatggtgtgcctatcggaaaggctgtgagcaattcttgggcctacgtcatggatctcaatcaacaactcgttccagttggtgtcatgggagaagctgtcgttattggagacggccttgcccgaggatatacagatcccgccctggattgcaaccgctttgtgcatatcactatcgatggcaaacgcgtgcgcgcctatcgaactggtgaccgcgcgcgttatcgacctaaagatggcgaaatcgaattctttgggcgtatggaccgacagctcaagattcgtggtcatcgtattgagcccgccgagattgagcatgccatgcttggccacaatgacatcgttgatgtagccattgtcactcgccatcaagatggtgcaggcttagaaatggttgcctttgttacagcccacactaacaagtctatcgaacgcaatgaagccaccaatcaagtagctggatggggggaccacttcgaatcgagtacatatgcagagctcgacacccttgtcaagtctgatgttggcaaggactttgtcggctggacgaacatgtatgatggcggcgcgatcgatcaggccgagatgcaggaatggcttgacgataccatacagacgattgttgatggtcagcctgctggtcatgtctttgagatcggtactggtaccggtatgatcatgtttggtctcgggaaacagggactgcaaagctacgtcggccttgagccctcaacctcggccactacgtacgtcaacaggaagatcaagaccgctccaacggtagctggcaaagccaaggtatatgtcggcactgcaatggaggcggctcaactcaatggactccatccggaagttgtcgtcatcaactctgtggctcaatacttccctacgccagaatatctcctcgaggtcgtcggtattctcactcagatgccaggtgtcaaacgcttgttctttggagacatacgatcgtatgctactaacaggaaattccttgcagccagagcccttcatatgctagggtccaacgcgaagaaacatgacattcgccggaaaatggctgagttggatgaattcgaagaagagttgattgtcgatccttctttcttcactggtctggtcagccgactgccaggccaggtcaagcatgtggagattcttccaaaacaaatgatcgccacaaatgagctcagcgcgtatcgttatgcagccgttgttcatctagctcttcccgaagagcagcacatagcgaaaatcgaaaagggcgcctgggtcgacttcacagccaccaagatggatcgaagcgctcttgttcatcatctgcagagctcgtcaaacgctgaaattgtagctatcagtaacattccattcagcaaaactaatttcgattgtcatcttctcgcatctctggatgaggacgaagaacactcgcttgacggatccgcctggatcaaaactattcattccagcgccgaacagtgtccatcgctatccgcaaccgatctcgtcgaagttgctaaagaggtgggcttccgtgtcgagctcagctgggctcggcaaaagtctcaaaacggtgcacttgacgctatcttccaccaataccaatctcccaaagaaggtagccgtgttctaatacagttcccgactgacgaccagggtcgatcgatggagtctcttacgaaccgaccgttacagcgagttcagagccgccggatcgaaacacagattcgtgagcgactacaggctgtgctaccatcatacatgattccagctcggatcgtggtgctaaatgagatgccagtcaatgccaacggcaaagtcgaccgcaaggagctgacgcgcagagcgaaggtggtcccaagaatcgaaacagctgcggagcgtattcaaccccgaaatgaagtcgaagcggttctgtgcgaggaattcagtgaagtcctcggcgtcgaagttggtgtcacggacaacttcttcgatcttggtggacactcgctcatggctacgaagctggctgcacgtactgggcgccgacttgatgcaaaggtgtctgtcaaagacgttttcgaccacccagtactagcggatcttgccgctgctattcagcgaggctcgactccccactcggcgatcgttactactgagtactctggacctgtagagcagtcatacgcccagggccgcctttggttccttgaacaactcaatttcaaggcaacgtggtatctcctaccgcttgcggtgcggattcgtgggccactcaatatcaaggcccttaccacggcgttacatgcgctagaacagcgacatgagactttaagaacaacattcattgagcgggatggtgtgggcaagcaggccgttcagccatttcagccgaaggaactcgaaatcgtcgacatagcggccgaccaccagggcgactaccttaaagtgctacgtgacgagcagactaccatgttcaatctagcaactcagcctggttggagggtgactttacacagagtggatcaaaacacgcataatctttccatcgtcatgcaccacatcatttcagacggctggtcagtcgatgttctgcgccacgagctgaggcagttctatgctgctgccctccggggtcaggatcccctcgcgcatatcagcccgctcccaattcaataccgcgacttctcgctctggcaaaagcagccagaccagatcatcgaacatgcaaaacaacttgagtactggaccaagcaactggcagacagctccccagctgagctcccaactgatttaccccgcccggccgtactgtcagggaaagctggcgaagtggccctttccgtcaagggcccgctatatgagcgtctgcaagctttctgcaagactcatcagacaactgccttcgccacactcctagcagccttccgtgcaacacatcatcgccttacaggagccgaagacgctaccatcggcacacctatcgccaaccgcaacaggcccgaattagagaacctgattggcttcttcgtgaatgctcagtgtatgcgcattactatcgatggagacgagactttcgagagtcttatacgtcaggtccgagccactgcgacggctgccatcgcaaatcaagatgtcccctttgaacgtatcgtgtctaccatgcaatctacctcacgagacacgtcaaggaatccgcttgtacagctcatgttcgccctccactctcaacaggacctcggaaaaatccaactagaaggctgcgaaacggagcctattccccgagctgtacgcactcgcttcgatctcgagttccatctctatcaagagcaagggagcctaggcggcattgtgtactttgccaccgatttgttcgagcctgagagcattgaggggatggtttccatttttaaagaaatcctcgctcgagctcttgaccaaccccaaaccccactggcgcttctaccgctcaccgatgggctggctgaacttcgcaggagggggctgcttgagattgaaaggcccagctatcctcgcgagtcgagcgttgttgacgtcttctgtagccaggtagcggcttctcccaacgcaaccgctgtgaaggactcgatttcacagctcacttacgctcagctaaatgagcaatctgacaaggtcgctgcttggctacaccagtgcaaccttccaactgaaactttggtcgctgtgctagcgcctcgatcttgccaaacagttgtggccttcttgggtattctgaaggccaacctagcatatcttcccctagacgtcaatgttccggcagctcgcattgaggcaattctctcagaagtctctggccacatacttgtcttacttggatctcatgtttctgctcccaagattgagctcgctgatgtcgaattcgtcaaaattgacaacacagtcgagcacaatttgccgggccgcattggatctgctccatctgccacgagcctcgcctatgttattttcacatctggatcgactggcaagcccaaaggtgttaaggtagagcaccgcggtattgtccgcctcgttaaagagagcaatgtagtagcaaaaatgccacaagctgcgcgcattgctcacttgtcaaacattgcctttgacgcggctacgtgggaattatatgctgcgttgctcaacggcggcaccctcgtctgtatcaactatttaaccacgctggatagtaaagcactcgaggccgtgtttgagcaggaaaagatccaagcggctatgcttccaccagcactgctcaaacagtatttggttaacattcccgcagctatcggtgcactagaagtggtccttgtcgctggtgaccgtttcgatcgacgcgatgctgcagccacgcaggctcttgttggagcaggcgtgtataacgcctatggaccgacggagaatacaacactcagcactatctacaatgtcgttcagggcgatgccaatgtgaatggcgtcccgattggacgccctgtcagcaactctggcgcctacatcatgaatatgaatcaggaactcgttcctattggcgtcataggcgagctggtcgtagtaggagacggtgtcgcccgaggatacaccgacccagccttggacgtcaaccgcttcgtcaacgtcactattgaaggccaaactatgagggcttataggactggcgatcgtgcccgctataggcccaaagacgcacagattgaattctttggccgaatggatcaacagatcaagattcgaggccatcgtattgagccagctgaggtcgagcatgcgttgctcaacaatgacttgcttcaggacgctgcagtcattatccgaaagcaacaaaatgatgagctggagatggttgcttttgtagaagcaaacagcaataagtcgatcgaacaagaggcgagcaaccaagtagaagactggggcgctcaattcgagagcaacgtctacgccgagatcgaggcaatcgatgcctctgctgttggtaacgacttcatgggttggacttccatgtacgacggcagcgcgatcgacaaggctgagatgcaggaatggctcgatgatactatgcagacaatacttgatggtcgaccagccggccgcgttctcgaaatcggcactggcacgggtatgatcctcttcaatcttggtgaagggttacagagctatgtcggtctcgaaccatctacctcggcggctgcgttcgtcaatcgcaggattcagacacttccagctttcgctggtaaagctgaagttcacgtgggtacagcgacagatataagccaacttcaagatctccgcccggaagtagtggttatcaactcggtggctcagtacttcccatcgcctgagtacttgtctaaggttttgtacgcactagcccaaattcctggcgtcaagcgtttgttctttggagacatgcgatcttacgccatcaacgaccagttccttgcagctcgcgccttacacaacataggtagcaaggctactaagagcgccattcgaagcaagatggtcgatctggaaaactctgaggaagaattgctcgtcgacccaaccttcttcaccaacctagcgaccgagcttccagaggttgagcatgttgagattctgccaaaacgcatgcaggctaccaacgaacttagcgcataccgatacgctgcggttgttcatattcgagacccagcaaggcaggcgcagacagtgcacaccattgatcctaccgcttggatcgattttagcgcatctcaaatgaatcgtactgctcttgccaacctcttgcaaaactcagcagatgctgcagctatcgctgtcagcaacatcccgtacagcaagacgatcttggcgcgccacattgttcagtcgcttgatgacgatctcacagacagcgatgatccacaagatgagcttgaaggagctgcttggatgtctgctatccggtccaatatcaaaacctgtgcatcgctgtccgccttcgaccttgcgcaacttgcccaggagaaaggcttccgtgtggagcttagttgggcaagacaacgaacccatcatggagctttagacgctgttttccatcattacaagtctaaccaggatggtggtcgtgtcctggtgcagttcccgactgatagtcgacctcgtctatcaggacaactcacaaaccaaccgctgcagcggctacagagtcgacgattggaggcacagattcgagatcagctcagcgctttacttccatcttacatgatcccgtcgcttatcgtgatggtcgatgagatgcccttgaatgccaatggcaaggtagacaggaaagccctagagcgaagggctcgcatggttcagaaagttgaaaagccagcttctgagcgagtcggtgcacgtaacgagatcgaagccgcgctgtgcgaagtattcgtagatctactcggcactgaggtcagcattactgacaacttctttaatcttggcggtcattcgctcatggccacaaaattggctgctcgaattagcagacgccttgacgcacgcatctctgtcaaggatgtgtttgactaccctgttctcgccgaccttgcgggcgccgttcagcgaggctcaactccacacaacccaatcgtcgcgacgccctactcagggcccgtcgagcagtcctttgctcagggccgcctgtggttcttggaccagcttaacgccggttcgctgtggtacatccagccaatcgccgtacgcgtacgcggttcgctcaatattggtgcgctgactacagcactcaatgcgcttgagaagcgccacgaaccgttgcgcacgactttcgaagagcatgacggcattggtgtgcaagtcgttcaaccgcatcagccgaagaagcttagaattgtcgatacggtggctaactatcagggtgacttcatcagggctctacggaaggagcagcagactctattcaatctcgcgaccgagccaggctggagagtgtctctgctacgcattggggaggacgacaacattctctccatcgtcatgcaccacatcatttcagacggttggtctgttgacatcttgcgtcaagatctaaaactattctatgccgccgctctcaaaagccaggagccgcaagtagacgcgctcccaatccaatatcgtgactttgccttctggcagaaacagccggagcaggtagctgagcaccagcgacaactcgactactggattgaacaattgaaagacagcaagcctgctgagcttatcaccgattttccgcggccagaggtgctgtctggcactgctggcatcgtacagcttgccgtggacggccaagtctacgagggtctccgggctttctgcagaattcatcaaacaacgtccttcgtggtacttcttgcagcctttagagctgcccattaccgtctaacaggcaccgaggacgcgacaatcggttctcccatcgccaaccggaatcggcccgaactggagagcctcattggcttcttcgtcaatacccaatgtatgcgcattatggtcggagaggacgacacattcgaacgattggtacagcaggtccgatcaacgacaacagctgcatttgctaaccaggacgttcccttcgaacgaatcgtttcatccgtccagtcaacctcaagagatgcctcccgaaaccctttggtacagctcatgtttgcacttcattcacagcagggtatcggcctgatggaactcgaaggtgttgagacagagccaattgcaagagatgtatcgacgcgcttcgacatcgagttccatctttaccagaaggaagagagcttacacggtgttgtccactttgctgccgacttgttcgagcctgagactattcaaggcttggtctccgtcttccaggaaattcttcgccgaggactcgagacacctcgattgccaatcagcattctgcctcttgataacaacattccggagcttctcgtcggtatgctcgatgtcgacactccagagtatcctcgcgattcaagcgtggttgatgtgttccgcacccaagttgctgccagcccggatgcgatcgccgttaaagattcaacttcgcagctcacctacgctcagcttgatgaagaatccaacaaagtggctacatggttgagtcaaaggcagctggctcccgaaacgctggtaggcgtccttgcgcctagatcgtgcccaacaatcgttacattctttggtatcctcaaggccagtctggcgtatctcccgctagacgtcaacgtaccatctgctcgtatcgaggcgatcctctcggcagtccctgaccataagttggtcttccttggtgctgacgtccccgatccagaggctccacttgtcaacgtggagctggtgcggatcgacgacatcttacgccaaagcattcacgcttcgaatgcagggcttctagcaaatcaccccttagcaactagtcttgcctacgtcatgtttacatctggatctacaggcaagcctaagggtgtcatggttgagcatcgaagtattgtacgcttggtaaaggaaacgaacctagtcccagcagtagaggcagtttcctcagtagctcacatctctaatgttgctttcgatgctgcaacttgggagatatacgctgcgctcctaaatggcggaactactgtttgcattgatcacattactgtgttggatcctgctaaactagctctcgtcttctcaagcgagaagatcaaagctgcgttcttctcaactgctttgctcaagcagcggctctacgaagagccatctactatcactggactcgatcttttatatgctggcggtgagagaatgaggcctcaagacgctcttaagacgcgagaactagttcgtggtagcttctgccacgtctatgggccgacagaaaatacaacattcagcactgtctatcctatgggggtagaagaacgctgcgtcaacggactacctatcggccgcgcagtcagccattcaggcgcagtgatcatggatgccaatcagcgcctcgtgccgttaggggtgatgggcgaacttgttgtcacaggtgatggtctcgcccgaggatacaccgatcccgctctgaatcgtgatcgcttcgtggaagtcaatatccacggtcaggtcctgagggcatatcgcacaggcgaccaagcccgctatcgacccaaagatggccagattgagttctccgggcgtatggacagacagctgaaaattcgaggccatcgtatcgagccagctgaggtcgagcacgccatacttagccacgacgatatccgaaacgcagttgtggttactcgacaacaggaaggccaagatctggaaatggtcgctttcgtctctactcccaacgatcaaaccgtagaacgcgacgaagctaggaatcaagttgaggactggggggctcaattcgagagcaacgtttacgccgagatcgaggagatcgactcctctgccgttgggaatgacttcatgggctggacgtctatgtacgacggtactgcgatcgataaagcagagatgcaggagtggctcgacgatactatgagaaccctccatgacggccgagatcctggccacgtcctcgaagttggtacaggcacgggcatgatcctattcaatctcggcaagggcctgcagagctacgtcggcctcgagccgtcgacttcggcagctgcattcgtcaatcgcaagattgagactatctcatcattggcgggtaaggctaaagttgagattggcacagcaaccgacgtaggccagctcaagaacctccgctccgatttggtcgttattaattcggtagctcaatacttcccttcccccgagtatctagtcgaagcagtaactgctctagtccacatcccaggtgtaaaacgcttgttcttcggcgacatgcgatcctacgccatgaataagcagttcctggttgctagggctctccgtacgctaggagccaaggcaaacaaggacgatgttcgcaggaagatggtggagctagaggaattcgaagaggaactactcgtggatccagccttcttcacaggcctcgcaaactggctgtcagaagtcgaacatgtcgagattctacccaaacagatgacatctaccaacgagctgagctcataccgttatgcagccatcgtacacctacggcttccaggccaggaggcacaaccagtcgtgacagtcaatcaagacgcctgggttgacttcggaggatccaagatggatcgacacgctcttcttcaccacctacaaagctcaccaaaggccgaaactgtagccatcagcaacatcccctatagcaagacgatttatgagcgccatgtcctcgcatctttggatgacgatgaagtcgaggactcgttagatgggtcagcatggctatcggctgttcgctctaccgccgaacagtgcgcgtcactctccggagtcgacttagttcaaatcgccaaggaggccggcttccgcgtggagctcagctgggcgcgacagaggtctcagaagggtggaatcgacgcggtcttccaccactacgagtcagtgcacgatggagctcgcgtcatggtcaagttcccgacagatgatcaaggccgagcgctcgattcgcttgcgaacaggccgctgcaacgactccagagtcgacgaatcgaggtgcaaattcgggagcggctacaagctgtactgccgtcctatatgatgccagtccgcattgtagtcttggacgagatgcctatgaatgcgaacggcaaggttgacagaaaagtgcttacccgcagagctaagatgatttcgagggtcgagacaaccgctgaacgcgttgggcctcgcaacgagatagaggctctcctctgtgaggagtttgctgaagtgcttggtgtcgaggttggcattaatgacgacttcttcgatcttggcggacactctctcatggccacgaagcttgcagctcgcagtagccgtcgcttcgatgcgaaggtctctgtcaaagacgtgtttgatcatcctatcctagcggacctagcagcttcgattcagcgaggctcaactccacacaaccccatcctcgcaacacaatatagcgggcctgtggagcagtctttcgctcagggtcggctgtggttccttgaacagctgaacgtcagttcaacatggtatctgcaaccaatcgcagtgcgtatgcgcggaccgcttaagattgaggcgctcgcggcggcgtttcacgctctggaggagcgtcacgaaaccctgcgaacgacgtttgaagagcacgacggcattggtatgcaggttgttcagccacatcgccccaaagaactcagagtgattgatgtacaggctgagcatgatggcgattatactcaggctctgcacacagagcaaacaactacgttcaatttagaaacggaaccaggatggagggtatcggtgtttcgcctgaacgaagatgacaacatcctctctatagtgatgcaccatatcatctctgatggttggtcgttcgatatcctgcgtaaggagatcagagagttttacaacgccgcgctcaagggcaaggaccccttggcgcaaatgagccccttgcatatccaatatcgcgacttttccgtttggcaaaagcagctgaatcagatcaccgagcataaacggcagcttgattactggacgaagaacctagccgacaatactccagccgagctcccaaccgatctgcctcggccagccgttctatccggtaaggctggagtcatccagctctctattacaggtccagtctatgatcgtctccgcgcgttctgccgagtccaccagaccaccttattcacggtgctcctcactgtatttcgagccacccactatcgcctcactggagcagaggatgctacgattggtacgcctatcgctaatcgtaacagaccagagcttgagaacttgatcgggttttttgttaacactcagtgcatgcggattaccgtagaagaggaggacacgttcgagacactcatccaccaggttcggactacaactacagccgctttcgccaaccaagacgtaccttttgagcgaattgtgtcagccctactcccaggctcccgagacacgtcccgcaacccgctctctcagatcatgtttgccgtacattctcagaaaaacatcagcaagatcgaactggacggcctagagagcgaggccatttcacgagccacatcaactcgtttcgatctagagttccatcttttccaggaagagaagggcctaggcggcattgtattgtttgcggcagatctgttcgagccggagacgatcgacagcctcgtcttcgtcttccaagagatcctccgccagagtctcgagacacccaagactccaattgcggtcttgcctcttaccaatggtattgcgcagcttcgcagcatgtgtgtgctagatattgagaagaccgcctaccctcaagactccagcgtcatcgatatcttccgccagcaggttgctgcccgcccggatgccacggccgtcacagattctacctctcagctcacctacgcacaactggatctccactctgacgagctagccagctggctgcgtcagaaaaagatggcacccgagactttggtgggtgtgctagcaccacggtcttgccaaacgatcgttacctttcttggtattttaaaggcgagcttagcctatttaccgctagacgtcaaagtgccggttgcccgcatagaggccattttgtcgtccatttcagggcagaaactgattctgcttgggcaggacgtacctgtcccagaaatccagctcccagacgtcgatgtcgtaccaatcagtgaaatcttaggccgctctgtcccttctcgtgctacagataagagtttaggaccattggcaagaaatcttgcgtatgttctgttcacatctggatccacaggcaagcccaagggtgtcatgatcgagcaccgtagtattgtgcgccttgtcaaagagacaaatcttatctctaagctaccaaacgcgcctcgcacggcacatctcaccaatctcgtctttgacaactctgcatgggaaatttactccacccttctcaacgggggaacgctagtctgcatcgactatgccaccgttctggatagcaaagccctcgagaccgtgttcaaggagcaacgcattcagacatctctgatgcctcctgcgctacttaaagagtgcttagccaacatgcctactatgttcgatgacgtagaggtgctctacgcgcttggagatcgattcgacaaacaggatgccatgaaagcgcgctcgatagtcaagaccgccgtctacaacgcctatggtcccacggaaaacacggtcatcagtactatctacgagattgccaaggacgattcgttcgtgaacggtgttcccatcggtcggagcatcagcaactccggagccttcatcatggactcccggcaacagctcgtccccgttggcgtgctaggcgagctcgtcgtttctggcgatggccttgcgagaggatatactgatcccacactggatgtaaatcgcttcgttgaggtgactgttgatggccaacatgttagagtataccggaccggtgatcgcgtacgcttccgtccaaaggatggtcagattgaattttttagtcgcatggatcagcaagtcaagattcgaggccatcgtatcgagccggctgaggtagagcacgttattctcaccaacaagattatccgtgatgcggctgttgcaatccggcgacctgagggtcaagaaccagaaatggttgctttcgttactacccatgaaaatacttctattgagaagcagtcagtcgaggaattcgcagcacggatcgagaatgaagtccgtcgctggatcaagaccttacttccgctctacatggttcctacacagattgttgtattggatcgaatgcctgtcaatgctaacggtaaggttgacaggaaagagctcgcgcaaagagcacaaaccctacagaagagcgaggccggttcccttccttccgtgagagttcctcccaccaacgacatggagaggatattgtgcgaagagtttgccgacgttctcggcgtggaggtcggcattaccgacaacttcttcgactttggaggacactcactcatggcaaccaagctcgcagcgcgtattagtcgccgcgtgaacgcccgagtatccgtcaagagcgttttcgaccaccccgtccttgttgaccttgcatccactattaaacaagactcaatcatgcacaaacctatcccacagaccgcctacaccgggcccgtggaacagtcctttgcccaaggccgtctctggttcttagaccagcttaacttcggtgcctcgtggtacctcatgcctctcgcgctacgcttgcaaggatctcttcacgtcaagtccctcactactgcgttgtttgcactagaacagcgtcatgagaccctgagaacaacatttgaggaacaagatggcgtgggcatccaaattgtacaccctgccaacaagaaagaccttagaatcctggacgtatctaaagagcaaaacagcgactatgctaaagtcctgcacaaggagcgcacgatccccattgatctgacttcggagccaggttggagggtatcgctcattcgcttgggcgaagacgatcatatcctctccatcgtcatgcatcacattatctcagatggatggtccgtggatgttctgcgccaagaactgaagcaattctatactgctgcgctcaagggtcaagatcctctggcgcagattgacgctctgccaatccaataccgcgacttctcattgtggcagaagttgccagatcaagttgctgagcaccaacgacagctcgagtactgggccgagcagttggcagataacactccagccgagctcctgaccgatctaccccggccggacgtcctatctggcaaggctggagccgtacaactcactatcgatggtccggtgttcgatcagctccaggcgttctgccgagcacatcagacaacaatgttcacggttctgctggcagtcttccgaacaactcattaccgcttgacaggcgctactgacgccactatcggtaccccgattgccaaccgtaacaggccggaacttgaaagattggtgggcttcttcgtcaatactcaatgtatcaggatcacggtagacgtggaggatacatttgaagcattggtacgacaagtccattctacgtcgacgacggcctttgccaatcaggatgttccgttcgagcgaattgtgtccacaattctaccaggctcgcgagacgcctcccggaatcctcttgctcaactcatgtttgccgtccattctcagagggatatcagtaaattccagcttgaaggcctagacacgaagcctatccccacggctgcatccactcgctttgacattgagttccatatgtttcagcaggcagaacgcctttctggaagggttcttttcgcagaggatctgttcgaactagagactatccaaggaatggttgtaatcttcaaagagattctccgaagaggccttgaaacgccacagaccccacttgcggttctcccactcactgatgggctggcacatcttcgcagtcaaggcctacttgagattgagaggccagagtatccgcgcgactcaagcatgatcgacgttttccgtgctcaggttgccgcatgccctgacgcgattgcggtcaaagactccacctcacagcttacctacagtcaactcgacgaccaatctgataagatcactgcctggcttctccaacgcaaaatcccagctgagagtttggttgctgtatacgctccaagaacgtgtcaaaccatcattacattctttggtattctcaaggctaatctagcctaccttccattggatatcaatgtcccagccgcccgtattgaggcaatcttatcaaccatatctggtcacaagctagtactgcttgggtctcaagtctccgctcctgcggtacaattgaaggacgtcgaatatgtttggattgatgaagccatggctgagactgttcgtacatgcaccagccccgaaccttctgccacaagtcttgcatacgtcatcttcacatccggatctacaggtctacccaagggcgtcaaggtcgagcaccgtggtgtcgtacgtctcgtcaagcagagtaatgtggtagcaaagatgcctcaagcagcacgcgttgcccatctatcaaatatcgctttcgacgctgccacgtgggagatctatgctgcgctccttaacggcggctctctcatatgtattgactatttcactacattggatagcaaggagcttgaagccgtgtttgcacgagaaaaaatccaagcggccatgcttccgccggcgctgctcaagcagtgtttggtcaacatccctgcgactatcagcgccttagacgtggtacttgcagcgggcgaccgtttcgacaggcgcgacgcggcggcgacacaagcgctcgtcggaggctgtgtctacaacgcgtacggccccaccgagaacacgactctcagtaccatctacaatgtggtcaaaggcgatgccaacgtcaacggagttccaatcggtcgccctgttagcaactcaggtgcctacatcatggatcccaatcaacagctggtccccaagggtgttatgggagagcttatcgtggtaggagacggagtcgctcgaggatataccgatccagcactagatgtcaatcgtttcattgagatcgcgattgatggtgatcaggcggtgcgcgcctatcgaacaggtgatcgcgctcgttaccgacctaaagacggtcaaatcgagttcttcggccgcatggaccaacaaatcaagattcgtggccatcgtattgaaccagccgaagtggagcacgccgtacttgataacagtatggtgcaagatgctgccgtaattactcgcaagcaagatcaggagctagagatgatcgcttttgttactacacgtagcgataaggaaattgacaacgacgaagccagcaaccaagtcgaagattggggtaaccagtttgagagtaacatatatgctgagatcgaagagatcgattcctctgccattggcaaagacttcatgggctggacgtccatgtacgacggtagtgctatcgacaaagacgaaatgcaggagtggctagacgacactatgagcacactgctcgacggtcgacaaccaggccacgtactcgaaatcggtactggtactggcatgatcttgttcaacctagccgagagaatgggattgaagagctacgtaggcctcgatccctcggagaaggcaacctcattcgttaaacaggccatcaagtctcgcccatctctggcaggcaaggctgaggttcacgtcggcacagcaacagatgtggctcgaatgcgagatctgcaccccgaagtggtggttatcaattcggtagctcaatactttccatcgcctgagtatctggccgatgtcgttggcgctttggttcgcattccaggcgtgaaacgactcttcttcggcgacatacgatcctacgctactaataatcatttccttgcagccagagccctacacaagctaggagaaaaggcaactagggatactgtacgaagcaaaatggctgagctcgaaggctacgaggaggaactgcttgtcgacccaacattcttcaccagtctaacggccaagcttcacggccaggtcgagcacgttgagatcctacctaagcgtatgcaggccaccaacgaactcagcgcataccgatacgcggctatagtctacatccgtgatccaaaacgagcgcagactgtgcagacggtcaaatcggacgcctgggtcgatttcagcacctctcaaatggaccgcagtgtgctcgtcagtctcttacagagctcagatgctgaagctatcgctgtcagcaatattccctacagcaagacgatcgtggcgcggcatatcgttgagtcactcagcgcagaggattcacaagagatgctggacggccctgcttggatctcagcagtccgctccagcgctgaacagtgcgcatccttgtctgcgatcgaccttgtacaggttgctaaagagaacggcttccgagtggagctcagctgcgcacgacagcggtctcataatggagcgattgatgcggtattccatcactacaagcctgcgcaagaaggtagccgtgtcttgctacaatttccaaccgacaatcacatccgggcaggctcgcttacgaaccgaccactacaacgtctcgagagtcgaagggtggagacaaaactcaaggaacacctttttagtgtgcttccatcgtacatgattccatcacatattgtgatggttgaccagatgcctctgaatgcgaacggcaaggttgaccggaaagccctggcacaaagagctgaagcagttctcaagatcgagaaaccagcttctgagagagtcagtgcacggaacgaagtggaagctgtactgtgtgaagagttcaccgatgtccttggtgtggaggtcggcattaccgacaacttcttcgacctgggcggacactcgctcatggccaccaaactcgcagcccgtatcagcaagcacctcgacgctcgcgtctctgtcaaggacgtttttgattaccctgtcgttgctgatctagcagcgtcaattgaacgaaactcgatccctcataaccccattccctcgaccaactactctggacccgtggagcaatctttcgcgcaaggccgactttggttcctggatcaactgaatatgggcgtatcggaattatatctaatgcctcttgctctacgcctgcgcggacctctgcgcgttgacgccttcgcagctgcagtatctgctctcgaggcacgccatgaaactctccgaacaaccttcatggatcacgacggtgtaggcatgcaagtcattctgcccagtaacagcaagaaactgagagtcattgacgcgtccgagaacgactatatagacatcctgcgacaggaacggacagctccattcaatctcacgaccgagccagggtttaggatcgccctcttgcagctgggtcaaaccgacttcattctgtcaattgtcatgcaccatatcatatatgacggttggtctattgatgttctatgcagagagcttggccgattctatagcgctgcactacagggccaggatccattggcgcaagtgagccctctgcctatccagtaccgagatttctctatctggcaaaagcggccagagcaagtggccgagcatgagcgccagctacaatactggactgaacaactggcagatagctctccagctgagcttcttacggatctaccccggccattggtgccaaccggtaaggccggtatcgttcaactcacgattgagggcgcagtctacgagcgccttcgagccttttgccgtgttcatcaaacgacctcgttcgctgtactcctcgcagccttccgtgcgacccactaccgtctcacgggcgctgaggatgctaccatcggctctccaattgctaatcgtaaccgcccagaactagaaagtctgattggcttctttgtcaatacccagtgtatacgcgtgacaatcagagaggacgataccttcgacaaattggtgcagcaagtccgggcaacgacaacagccgcgcaggtcaaccaggatgtcccattcgaacgcatcgtctcagctctgatgcctggctcaagagacacgtcccgaaatccactagtgcagctcagctttgctcttcactcacagcatgaccttggaagaatcgatctccaggatctgacaggagaagctcttcccacaccagtgttcaccagactggatgtagagttccatcttttccagcaagctgagaagttcggtggtagcgtattgtttgcaacagacttgtttgagccggagactattcaaggactggtctccgtcttccaggaggtcttacgccgaggacttgagcaaccccaaacgcctattgcagttctgccccttgacaacgcgtccgaggatcttcggagcatgggtctgcttcaaatggagagaaccaactatccacgggactctagtgtggttgatgtcttccgtgatcaggtggcagccaatcctagagcaatagccgtcaaggattcagtcttagagctgacctacgctcagctggacgagaaatctgaccagttggctgcctggctctgccaacataacattccggcagagacaatcgttggcgttctggctccgagatcttgcgagacaattattgccttcctcggaatcctcaaggccaacctcgcatacttgccattagacgataatgttccagctgctcgcattgagactatattgtcagcagtccctggccacacattagtcctactcggctcacatgtggctgctccaagcattggattagcagatgctgaattcgttaatatcaatcatactttaggccacagtttgcaactcaacagcacatgcgccaagttgcagccctccgctacaagccttgcatatgttatctttacatctgggtcgacaggcaagccaaaaggcgttatgattgagcacagaagcattgtgcgacttgtcaaaaacagcaataccctcgccaagctcccacgagccgctcgtgtcgctcatcaattcaaccttgccttcgatgcagcaaactacgagatctatggtacactgctgaatgggggtgccctgatctgtgtcgattactccaccctcttggacattgatgctctcgtggccatgttcaagcgagagaaaatcaccgcatcctcactgtctcctggtttgctcaagcagtgtgtgaacagtgcacccgaaatgctcaaggctttacaggtgatctacacaggtggagaccgactcgatggtcgcgatgccattgagttgcaagcacttgttcccggaggcgtttacaacatgtacggacctaccgaaaacacagtcatcagcacgctttacaatctcggcgacaagcattcgtatgtgaatggcgttcccattggaacaaccgtcagcaattcgggagcctacgtcatggatgccctgcaacagctcgtccctgtcggagtaatgggagagctcgtcgtcactggggatggacttgctcgagggtacactgatccggaactagaccgcaaccgattcatcaaggtcaacattgatggtcaggtcgtcagggcgtaccgaacaggcgatcgcgtccgctaccgaagaatagacggtcaattagaattcttcgggcgcatggatcagcaaattaagattcgaggcttccgtatcgagacggcggaagttgagaacgccatgctcagtcacagcgcagttcgcaatgctgctgttgtcgtccctacccaagacattcaagagaagggaatgattggtttcgtggtgattgaaaacaatacacccaagaacgaggagagcaaggaagaacacttgctacaaactgaattggcgatcctcaaccggatgaagagcatccttcctccttacatgctcccatctcgcatcatcatccttgatcagatgccttcgaatttcaatggaaaggtcgatcgtaaagagcttgatcgcatggctcagagcgtacctagacagaagactacggcagggcgcatagttccccgcaatgaattggaagcttcgctctgtaaggagttcgctgaagtgctcggcgttgaggtcggcatcactgacaatttcttcgacctcggtgggcactcgctactggcaaccaagctcgcagctcgcattagccgcaggctggatactcgcgtgtctgttaaagacgtattcgatcagcctgtgcccgcagatctagcactcaaggtttcgtcttacatctcccaaggtcatgcaatggacaacggaaccttgtcgacaacgaacagcatccccttccagctactacattttgaagattcgcagaaatttatcgaccgcgacattgtcccgcaacttgctcatcagtcagctaaaattgtggatgtctatcctgttacgtggatacagaagcacttccttgttgatccagcaacaggacttccacgtacaccatcactcttctttgtcgatttcccagccaacgctgactgcgacaaaatttgcaatgcgagccggtctctcattcagcttttcgatatcttcaggactgtctttgttcaggctgccggcaatttttaccaagtcgttctggaagagcttgacatacccatctcggtcatcgaaaccgaagacatcagtactgcaactcgcgtcctgaaggaacaggatcaacaaaatccgctccaattcggacaaggattcttacgctttgcagtcgtgaagacgaggtcagctgtgcgcttggtacttcgcatctctcattgcttgtacgatggcttgagtttcgagcatgttgtgcaatcacttcatgctttgtataatggcgaccgcatcccaacacagcccaagttcgttcagtatgttcagcatctgactgacagccgcaaagaaggttacgatttctggctatctgtcctggaggagtcctcgatgacagtcgtagagactggccgtcgcgctcaacaactatcatcacctgagggtgcttggttcgtcgagaagattatcaaggctgttatcccagccaactcagatggtattacgcaggcaacagtatttaccactgcttccaccatcctgcttgccagaatgaccggatcaagcgacatcaccttcagccgactcgtatctgggcgtcaatctttgccgatcaatgaccaacatatcgtcggcccttgcacaaacatcgtccccgttcgtattcgcatgactgatggcactaatgcaagagagcttctcggcatggtgcaagaccaatacatcgacagcttgccatttgaaacgctagggttcgatgacatcaaggagaactgcactaaatggccagcgtcgactacgaactacggctgctgcagcacattccagaacttcgagatgcagcctcaaagtcaagtccaggacgaacgtgttcgattggctggtttgacaaatttcaaagatgcagaactactaaatggcgctaccgctacaaacaagagagttctagatgacgtaccaatgcatgagattgatatgattggaatccctgagccggatggacttcatgtacgagttgtccttaccgctagcaggcagattttcgaggaggaggttgtggaccgcatgcacgaagagttctgcgatatcatcttgggtttgaacaagatcttgcaaaaatag

SEQ ID NO: 37 - protein, 13041 aa, Curvularia clavata
MASDINTHPEGATKFWQQHFDGLNASVFPALSSHLTVPRPNAQTAHRISYSTLAKQKWDNTSLCRAALAILLARYSNASEALFGVLVEQFLPSNGEQASTEESPQSILPIRIRLDLEEAGLGLLQAINTLDASLREWKHIGLDAIRGTGEYGSAGCEFQTVLAVTTGKTPRTHRLASCTDRALLLDCRMDDDSATLLARYDPSVIDDLQVARFLKQLGHVIEQLRVQAVDLPLWELGIVTQEDSAEIQKWNSQQLQFSQECIHDVFANRVVDTPQKIAVSAWNGELTFAELDSFSSCLAQHIQSLELGDAKAIPLCFEKSKWAIVGMLGVLKAGRAFTLIDPSNPPARARQICRQTAATISIASPYQCDMMRALVPDCIVVDDDFFKSLAFDTDQFQPTATPQTLAYILFTSGSTGEPKGSMMEHHGFVSCCLEFGAALGINSNTRALQFASYAFGACLLEILTTLMHGGTVCIPSDDERINDAPGFIRRANVNWAILTPSFIGAIQPTTVPNLKTLVLVGEAMPSDIRDVWASHVQLKNAYGQSESATICSVTEVTPATVEAHNIGHAVGARFWITDPNNPNKLAPIGCVGELLVESPGIARGYLIPLPADATPFIDTLPDWYPRTQPLDNFKFYRTGDLVCYRSDGTVVYLGRRDSQIKIRGQRVEIGEVETCLRQQLPSQLVPVVEAVSLSGMSKSMTLIAFLVGENTILEEDVYVLEGSAAQRISSKLRQIVPGYCIPSHYIRINHLPTTATGKCDRKALRAIGTKLLREAVEGMASQEEQESASLMTEGITLERIWFQSLGLKPNSTRHKSNFFNLGGDSIAAIRMVNMARAAGLLLSISDIFQNPSLAGLINVMQQSSTAQDAIPATEYSGPVEQSFAQGRLWFLDQLTTGASWYLMPLAVRIHGPLRVQALSSALHALEQRHETLRTTFEQQDGMGVQIVHPSSKRELRVIDVSGKQNGGYDQVLKREQTTPIDLAKEPGWRAALLRVGDDEHILSIVIHHIIYDGWSLGVLREELGDLYAAALRGPDPLAHMAPLPIQYRDFSVWQKQPQQVAQHQQQLVYWTKQLEDSAPAELLTDFPRPAELSGRAGEVRFTIEGSVFDSLLAFRRVHQTTSFAVLLAVFRAAHYRLTGTEDATIGTPIANRTRAEVEKLIGFFVNTQCMRIAVADDDTFASLVSQVWSVATAAFEHQDVPFERIVSALLPGARDTSRNPLAQLLFALHLEQDLDKINLEGLACETVPTPMATRFDVEFHLFQEDDRLNGVVNFSTDLFEPQTIHSLVSVFQEILRRGLDQPQTPIAHLQLTDGLEELRNAGLLDIKRIDYPREASVVDMFQKQVAACPNVTAVKDSTSQLTYAQLDQESDKIAVWLRKRNIPAETLIALLAPRSCDSVAAFLGILKANLAYLPLDVNVPAARIEAILSTVAGHKLVLLGRDVPLLGTQLADLELVRIGEALRGSSSGSVAADKAIRPTATSLAYVIFTSGSTGQPKGIMVPHRSLVNVIKQRPAYGNVAHMTNLAFDPSLFEMCTALFNGNTLICIDTLVALDATQLPTIFKQEAIRVAMMTPALLTRLLAQATDALHELEALYVLGDRFPPKDAARASELVKTAVYNAYGPSENSICTTLFHAATGAMCTNGVPVGRVINNSGVYVMDPKQSLVSYGVMGELVVAGEGLAIGYTKPELNEGRFLTLTMDGKPVRAFRTGDRVRYRPTDGQLEFFGRMDFQIKIRGHRVELAEVERVLNRHPAIKDAITLLRQHGSSAQDTELVSFIVLGEQKPVKPHRNATDHGGMEIEQLDQKLEANLRAMMQATLPSYMVPSRIIVLDHMPLDKNGKVDRRGLTGLTLSPAMETSSRVVVAARNEIEAVLCEEFAHILGVEIGVTDNFFDLGGHSLMATTLAARLARRLNASISVKDVFDQPIVANLAATIKRGSTPHNAIPPTKYSGPVEQSFAQGRLWFLDQLNLGAAWYHMPLAVRLRGPLHLEALTAALHALEERHETLRTVFEEQDGVGMQIVRPSSKTPLRIIDVSTKERGYAELLKQEQTTPFDLATELGWRVALLRQGKDDHILSIVIHHIISDGWSLDILCEELGQFYAAVLRGQDPLAQISPLPIQYRDFSLWQKQPEQVAEHHRQLEYWTTQLEGSVPAELLTDLPRPTIQSGKAGVIPITVNGPVYERLRAFSRAHQTTAFAVLLAAFRATHYRLSGVADATIGTPIANRNRPELENMIGFFVNAQCMRITVEQDDTFETLVRQIRFTATAAFANQDVPFEHIVSALMPDSRDTSRNPLVQLMFALHAYKDLGKIELEGYVAEPVHTTLSTRFDLEFHMFQETNHLSGYVLYATDLFEPESIEGMVSIFKEILARALDQPQTPLALLPLTDGLAELRRRGLLEIERPSYPRESSVVDVFCSQVAASPNATAVKDSISQLTYAQLNEQSDKVAAWLHQCNLPTETLVAVLAPRSCQTVVAFLGILKANLAYLPLDVNVPAARIEAILSEVSGHILVLLGSHVSAPKIELADVEFVKIDNTVEHNLPGRIGSAPSATSLAYVIFTSGSTGKPKGVKVEHRGIVRLVKESNVVAKMPQAARIAHLSNIAFDAATWELYAALLNGGTLVCINYLTTLDSKALEAVFEQEKIQAAMLPPALLKQYLVNIPAAIGALEVVLVAGDRFDRRDAAATQALVGAGVYNAYGPTENTTLSTIYNVVQGDANVNGVPIGRPVSNSGAYIMNMNQELVPIGVIGELVVVGDGVARGYTDPALDVNRFVNVTIEGQTMRAYRTGDRARYRPKDAQIEFFGRMDQQIKIRGHRIEPAEVEHALLNNDLLQDAAVIIRKQQNDELEMVAFVEANSNKSIEQEASNQVEDWGAQFESNVYAEIEAIDASAVGNDFMGWTSMYDGSAIDKAEMQEWLDDTMQTILDGRPAGRVLEIGTGTGMILFNLGEGLQSYVGLEPSTSAAAFVNRRIQTLPAFAGKAEVHVGTATDISQLQDLRPEVVVINSVAQYFPSPEYLSKVLYALAQIPGVKRLFFGDMRSYAINDQFLAARALHNIGSKATKSAIRSKMVDLENSEEELLVDPTFFTNLATELPEVEHVEILPKRMQATNELSAYRYAAVVHIRDSSERAQTVHAIKSSAWVDFSKSQMDRKALISLLQSSVNTEAVAIGNIPYSKTIMARHVVQSLDEDNADKDIAQDKPDKPTWISAVRSNAEHCPSLSALDLVQLGEEAGFCVELSWAQQRSHHGAIDAVFHHYQPAREGSRVLFQFPTDTYRRQSGPLTNRPLQRIQSRRMETQVREKLRAVLPSYMIPSLIVLVDQMPLNPNGKVDRKALERRAQAVLRVEKPTSERVGARNETEAVLCEEFTDVLGLEVGITDNFFDLGGHSLMATKLAARISRRLDARVSVKDVFDQPVIVDLAASIRRGSTPHNPITPTEYSGPVEQSFAQGRLWFLDQLNLGASLYLMPLALRLRGPLRIDALTAALFALEQRHETLRTVFKEQDGVGIQIIQPSQKKKLRTIDVSAGDFSEALHHERTAPFDLASEPGFRVALLQLEPSDHVLSIVMHHIIYDGWSIDILCQELGQFYAAAIQGQDPLGQVSPLPIQYRDFSVWQKQPEQVAEHERQLAYWIDQLADSAPAEFLVDLPRPPVLSGDAGLVHLTIDGPIYDRLRAFCRVHQTTTFAVLLAAFRATHYRLTGAEDATVGTPIANRNRPELENLVGFFVNTQCMRISVGDDDTFEQLVRQVRSTATAAFANQDVPFERIVSTLLPGSRDTARNPLVQLMFAVHSLKDLGKIQFEGLVGETIPTASFTRFDVEFHLFQEVGRLSGNVLFSTDLFEPETIQGMVSVFMEILRGALDQPQIPIAVLPLTDGLTELRNRGLLEVEQPQYPRDSSVIDVFRAQVVACPDAIAVKDSTSQLTYAQLDEQSDEVAVWLHQRKLPAESLVAVLAPRSCETIITFFGILKANLAYLPLDINVPAARIQAILSSVAGKKILLLGSDQAQPEIRLDDVEFVQINETIDHNMAKDNTTRSGPLATSLAYVIFTSGSTGQPKGVKVEHRGIVRLVKNSNVVAKMPEAACVAHLSNLAFDAATWEIYAALLNGGSLICIDYFTTLDSKVLEAVFEREQIRAAMFPPALLKQCLLNIPTTISALDVILAAGDRFDRRDAIAAQALVGGGVYNAYGPTENTTLSTIYNVVDGDTNVNGIPIGLPVSNSGVYVMDPNQQLVPLGVMGELVVVGDGVARGYTDPALDVDRFIKVEIDGQIVRAYRTGDRVRHRPKDGQIEFFGRMDQQVKIRGHRIELAEVEHVILDNSLVQDAAVIVHKQADQEIEMIAFAIVRGDNDSKHPEKDILDRVKALLPSYMVPAQMVLLNSMPLNANGKVDRKELAKRAGTVPRSEMAYVAPERVPPRNEIETILCEEYAEVLGVEVGVMDNFFDLGGHSLMATKLAARATRRLDAKLSVKDIFDYPILANLAAAVQRGSTPHNAILATTYSGPVEQSFAQGRLWFLDQLNVGSNWYLQPIAIRIRGSLNINALTTALHALEQRHETLRTTFEEEDGVGMQVVQEYDPIELRIMDIAADYDGDYTEALKGEQTTPFDLESEPGWRVSLLRMNDNDHILSLVLHHIISDGWSVDVLRQELKQFYAAALQGLDPLSGADPLPIQYRDFSLWQKQPEQVAEHERQLKYWVEQLADNSPATLLADRPRPSVLSGQAGSVPLSIEGQVYEKLQAFCRAHQTTSFSVLLAAFRAAHFRLTGVDDATIGIPIANRNRPELEHLIGFFVNRQCMRITVGEDDTFESLIRQVHSTATAAYANQDVPFERIVSSLLSGSRDTSRNPLVQLVFAVHSQKNLGKFELQDLTSEPVAGAISTRFDAEFHLFQEEERLNGVVYYATDLFDAETIQGVVSVFQEILRRGLNHPRTPIAALSLTDGLDNLRKMNLVHFKRTDYPRDSSMVDIFREQVATYPDVIAVKDSTLQLTYAQLDQQSDEIATWLRNKKMAPETLVGVLAPRSCQTIVAFLGVLKANLAYLPLDVNAPMARVETIMSSVPGSKLLLLGSDVPAQEIQLQNVELVRIEDTLGHAASAGTATTEPSPTSLAYVIFTSGSTGKPKGVMVEHRSVIRLVRKESNSMSKMSSRARVAHLTNIAFDVSAWEVYATLLNGGTLVCVDYFTSFDAKALGLLFEREQITAAMITPTLLKQCITIVPEALRKLSVLYTGGDRFDRRDAIATKALVKGPVYNAWGPTETTIVSTIYELADDDQFTNGVPIGKAVSNSWAYVMDLNQQLVPVGVMGEAVVIGDGLARGYTDPALDCNRFVHITIDGKRVRAYRTGDRARYRPKDGEIEFFGRMDRQLKIRGHRIEPAEIEHAMLGHNDIVDVAIVTRHQDGAGLEMVAFVTAHTNKSIERNEATNQVAGWGDHFESSTYAELDTLVKSDVGKDFVGWTNMYDGGAIDQAEMQEWLDDTIQTIVDGQPAGHVFEIGTGTGMIMFGLGKQGLQSYVGLEPSTSATTYVNRKIKTAPTVAGKAKVYVGTAMEAAQLNGLHPEVVVINSVAQYFPTPEYLLEVVGILTQMPGVKRLFFGDIRSYATNRKFLAARALHMLGSNAKKHDIRRKMAELDEFEEELIVDPSFFTGLVSRLPGQVKHVEILPKQMIATNELSAYRYAAVVHLALPEEQHIAKIEKGAWVDFTATKMDRSALVHHLQSSSNAEIVAISNIPFSKTNFDCHLLASLDEDEEHSLDGSAWIKTIHSSAEQCPSLSATDLVEVAKEVGFRVELSWARQKSQNGALDAIFHQYQSPKEGSRVLIQFPTDDQGRSMESLTNRPLQRVQSRRIETQIRERLQAVLPSYMIPARIVVLNEMPVNANGKVDRKELTRRAKVVPRIETAAERIQPRNEVEAVLCEEFSEVLGVEVGVTDNFFDLGGHSLMATKLAARTGRRLDAKVSVKDVFDHPVLADLAAAIQRGSTPHSAIVTTEYSGPVEQSYAQGRLWFLEQLNFKATWYLLPLAVRIRGPLNIKALTTALHALEQRHETLRTTFIERDGVGKQAVQPFQPKELEIVDIAADHQGDYLKVLRDEQTTMFNLATQPGWRVTLHRVDQNTHNLSIVMHHIISDGWSVDVLRHELRQFYAAALRGQDPLAHISPLPIQYRDFSLWQKQPDQIIEHAKQLEYWTKQLADSSPAELPTDLPRPAVLSGKAGEVALSVKGPLYERLQAFCKTHQTTAFATLLAAFRATHHRLTGAEDATIGTPIANRNRPELENLIGFFVNAQCMRITIDGDETFESLIRQVRATATAAIANQDVPFERIVSTMQSTSRDTSRNPLVQLMFALHSQQDLGKIQLEGCETEPIPRAVRTRFDLEFHLYQEQGSLGGIVYFATDLFEPESIEGMVSIFKEILARALDQPQTPLALLPLTDGLAELRRRGLLEIERPSYPRESSVVDVFCSQVAASPNATAVKDSISQLTYAQLNEQSDKVAAWLHQCNLPTETLVAVLAPRSCQTVVAFLGILKANLAYLPLDVNVPAARIEAILSEVSGHILVLLGSHVSAPKIELADVEFVKIDNTVEHNLPGRIGSAPSATSLAYVIFTSGSTGKPKGVKVEHRGIVRLVKESNVVAKMPQAARIAHLSNIAFDAATWELYAALLNGGTLVCINYLTTLDSKALEAVFEQEKIQAAMLPPALLKQYLVNIPAAIGALEVVLVAGDRFDRRDAAATQALVGAGVYNAYGPTENTTLSTIYNVVQGDANVNGVPIGRPVSNSGAYIMNMNQELVPIGVIGELVVVGDGVARGYTDPALDVNRFVNVTIEGQTMRAYRTGDRARYRPKDAQIEFFGRMDQQIKIRGHRIEPAEVEHALLNNDLLQDAAVIIRKQQNDELEMVAFVEANSNKSIEQEASNQVEDWGAQFESNVYAEIEAIDASAVGNDFMGWTSMYDGSAIDKAEMQEWLDDTMQTILDGRPAGRVLEIGTGTGMILFNLGEGLQSYVGLEPSTSAAAFVNRRIQTLPAFAGKAEVHVGTATDISQLQDLRPEVVVINSVAQYFPSPEYLSKVLYALAQIPGVKRLFFGDMRSYAINDQFLAARALHNIGSKATKSAIRSKMVDLENSEEELLVDPTFFTNLATELPEVEHVEILPKRMQATNELSAYRYAAVVHIRDPARQAQTVHTIDPTAWIDFSASQMNRTALANLLQNSADAAAIAVSNIPYSKTILARHIVQSLDDDLTDSDDPQDELEGAAWMSAIRSNIKTCASLSAFDLAQLAQEKGFRVELSWARQRTHHGALDAVFHHYKSNQDGGRVLVQFPTDSRPRLSGQLTNQPLQRLQSRRLEAQIRDQLSALLPSYMIPSLIVMVDEMPLNANGKVDRKALERRARMVQKVEKPASERVGARNEIEAALCEVFVDLLGTEVSITDNFFNLGGHSLMATKLAARISRRLDARISVKDVFDYPVLADLAGAVQRGSTPHNPIVATPYSGPVEQSFAQGRLWFLDQLNAGSLWYIQPIAVRVRGSLNIGALTTALNALEKRHEPLRTTFEEHDGIGVQVVQPHQPKKLRIVDTVANYQGDFIRALRKEQQTLFNLATEPGWRVSLLRIGEDDNILSIVMHHIISDGWSVDILRQDLKLFYAAALKSQEPQVDALPIQYRDFAFWQKQPEQVAEHQRQLDYWIEQLKDSKPAELITDFPRPEVLSGTAGIVQLAVDGQVYEGLRAFCRIHQTTSFVVLLAAFRAAHYRLTGTEDATIGSPIANRNRPELESLIGFFVNTQCMRIMVGEDDTFERLVQQVRSTTTAAFANQDVPFERIVSSVQSTSRDASRNPLVQLMFALHSQQGIGLMELEGVETEPIARDVSTRFDIEFHLYQKEESLHGVVHFAADLFEPETIQGLVSVFQEILRRGLETPRLPISILPLDNNIPELLVGMLDVDTPEYPRDSSVVDVFRTQVAASPDAIAVKDSTSQLTYAQLDEESNKVATWLSQRQLAPETLVGVLAPRSCPTIVTFFGILKASLAYLPLDVNVPSARIEAILSAVPDHKLVFLGADVPDPEAPLVNVELVRIDDILRQSIHASNAGLLANHPLATSLAYVMFTSGSTGKPKGVMVEHRSIVRLVKETNLVPAVEAVSSVAHISNVAFDAATWEIYAALLNGGTTVCIDHITVLDPAKLALVFSSEKIKAAFFSTALLKQRLYEEPSTITGLDLLYAGGERMRPQDALKTRELVRGSFCHVYGPTENTTFSTVYPMGVEERCVNGLPIGRAVSHSGAVIMDANQRLVPLGVMGELVVTGDGLARGYTDPALNRDRFVEVNIHGQVLRAYRTGDQARYRPKDGQIEFSGRMDRQLKIRGHRIEPAEVEHAILSHDDIRNAVVVTRQQEGQDLEMVAFVSTPNDQTVERDEARNQVEDWGAQFESNVYAEIEEIDSSAVGNDFMGWTSMYDGTAIDKAEMQEWLDDTMRTLHDGRDPGHVLEVGTGTGMILFNLGKGLQSYVGLEPSTSAAAFVNRKIETISSLAGKAKVEIGTATDVGQLKNLRSDLVVINSVAQYFPSPEYLVEAVTALVHIPGVKRLFFGDMRSYAMNKQFLVARALRTLGAKANKDDVRRKMVELEEFEEELLVDPAFFTGLANWLSEVEHVEILPKQMTSTNELSSYRYAAIVHLRLPGQEAQPVVTVNQDAWVDFGGSKMDRHALLHHLQSSPKAETVAISNIPYSKTIYERHVLASLDDDEVEDSLDGSAWLSAVRSTAEQCASLSGVDLVQIAKEAGFRVELSWARQRSQKGGIDAVFHHYESVHDGARVMVKFPTDDQGRALDSLANRPLQRLQSRRIEVQIRERLQAVLPSYMMPVRIVVLDEMPMNANGKVDRKVLTRRAKMISRVETTAERVGPRNEIEALLCEEFAEVLGVEVGINDDFFDLGGHSLMATKLAARSSRRFDAKVSVKDVFDHPILADLAASIQRGSTPHNPILATQYSGPVEQSFAQGRLWFLEQLNVSSTWYLQPIAVRMRGPLKIEALAAAFHALEERHETLRTTFEEHDGIGMQVVQPHRPKELRVIDVQAEHDGDYTQALHTEQTTTFNLETEPGWRVSVFRLNEDDNILSIVMHHIISDGWSFDILRKEIREFYNAALKGKDPLAQMSPLHIQYRDFSVWQKQLNQITEHKRQLDYWTKNLADNTPAELPTDLPRPAVLSGKAGVIQLSITGPVYDRLRAFCRVHQTTLFTVLLTVFRATHYRLTGAEDATIGTPIANRNRPELENLIGFFVNTQCMRITVEEEDTFETLIHQVRTTTTAAFANQDVPFERIVSALLPGSRDTSRNPLSQIMFAVHSQKNISKIELDGLESEAISRATSTRFDLEFHLFQEEKGLGGIVLFAADLFEPETIDSLVFVFQEILRQSLETPKTPIAVLPLTNGIAQLRSMCVLDIEKTAYPQDSSVIDIFRQQVAARPDATAVTDSTSQLTYAQLDLHSDELASWLRQKKMAPETLVGVLAPRSCQTIVTFLGILKASLAYLPLDVKVPVARIEAILSSISGQKLILLGQDVPVPEIQLPDVDVVPISEILGRSVPSRATDKSLGPLARNLAYVLFTSGSTGKPKGVMIEHRSIVRLVKETNLISKLPNAPRTAHLTNLVFDNSAWEIYSTLLNGGTLVCIDYATVLDSKALETVFKEQRIQTSLMPPALLKECLANMPTMFDDVEVLYALGDRFDKQDAMKARSIVKTAVYNAYGPTENTVISTIYEIAKDDSFVNGVPIGRSISNSGAFIMDSRQQLVPVGVLGELVVSGDGLARGYTDPTLDVNRFVEVTVDGQHVRVYRTGDRVRFRPKDGQIEFFSRMDQQVKIRGHRIEPAEVEHVILTNKIIRDAAVAIRRPEGQEPEMVAFVTTHENTSIEKQSVEEFAARIENEVRRWIKTLLPLYMVPTQIVVLDRMPVNANGKVDRKELAQRAQTLQKSEAGSLPSVRVPPTNDMERILCEEFADVLGVEVGITDNFFDFGGHSLMATKLAARISRRVNARVSVKSVFDHPVLVDLASTIKQDSIMHKPIPQTAYTGPVEQSFAQGRLWFLDQLNFGASWYLMPLALRLQGSLHVKSLTTALFALEQRHETLRTTFEEQDGVGIQIVHPANKKDLRILDVSKEQNSDYAKVLHKERTIPIDLTSEPGWRVSLIRLGEDDHILSIVMHHIISDGWSVDVLRQELKQFYTAALKGQDPLAQIDALPIQYRDFSLWQKLPDQVAEHQRQLEYWAEQLADNTPAELLTDLPRPDVLSGKAGAVQLTIDGPVFDQLQAFCRAHQTTMFTVLLAVFRTTHYRLTGATDATIGTPIANRNRPELERLVGFFVNTQCIRITVDVEDTFEALVRQVHSTSTTAFANQDVPFERIVSTILPGSRDASRNPLAQLMFAVHSQRDISKFQLEGLDTKPIPTAASTRFDIEFHMFQQAERLSGRVLFAEDLFELETIQGMVVIFKEILRRGLETPQTPLAVLPLTDGLAHLRSQGLLEIERPEYPRDSSMIDVFRAQVAACPDAIAVKDSTSQLTYSQLDDQSDKITAWLLQRKIPAESLVAVYAPRTCQTIITFFGILKANLAYLPLDINVPAARIEAILSTISGHKLVLLGSQVSAPAVQLKDVEYVWIDEAMAETVRTCTSPEPSATSLAYVIFTSGSTGLPKGVKVEHRGVVRLVKQSNVVAKMPQAARVAHLSNIAFDAATWEIYAALLNGGSLICIDYFTTLDSKELEAVFAREKIQAAMLPPALLKQCLVNIPATISALDVVLAAGDRFDRRDAAATQALVGGCVYNAYGPTENTTLSTIYNVVKGDANVNGVPIGRPVSNSGAYIMDPNQQLVPKGVMGELIVVGDGVARGYTDPALDVNRFIEIAIDGDQAVRAYRTGDRARYRPKDGQIEFFGRMDQQIKIRGHRIEPAEVEHAVLDNSMVQDAAVITRKQDQELEMIAFVTTRSDKEIDNDEASNQVEDWGNQFESNIYAEIEEIDSSAIGKDFMGWTSMYDGSAIDKDEMQEWLDDTMSTLLDGRQPGHVLEIGTGTGMILFNLAERMGLKSYVGLDPSEKATSFVKQAIKSRPSLAGKAEVHVGTATDVARMRDLHPEVVVINSVAQYFPSPEYLADVVGALVRIPGVKRLFFGDIRSYATNNHFLAARALHKLGEKATRDTVRSKMAELEGYEEELLVDPTFFTSLTAKLHGQVEHVEILPKRMQATNELSAYRYAAIVYIRDPKRAQTVQTVKSDAWVDFSTSQMDRSVLVSLLQSSDAEAIAVSNIPYSKTIVARHIVESLSAEDSQEMLDGPAWISAVRSSAEQCASLSAIDLVQVAKENGFRVELSCARQRSHNGAIDAVFHHYKPAQEGSRVLLQFPTDNHIRAGSLTNRPLQRLESRRVETKLKEHLFSVLPSYMIPSHIVMVDQMPLNANGKVDRKALAQRAEAVLKIEKPASERVSARNEVEAVLCEEFTDVLGVEVGITDNFFDLGGHSLMATKLAARISKHLDARVSVKDVFDYPVVADLAASIERNSIPHNPIPSTNYSGPVEQSFAQGRLWFLDQLNMGVSELYLMPLALRLRGPLRVDAFAAAVSALEARHETLRTTFMDHDGVGMQVILPSNSKKLRVIDASENDYIDILRQERTAPFNLTTEPGFRIALLQLGQTDFILSIVMHHIIYDGWSIDVLCRELGRFYSAALQGQDPLAQVSPLPIQYRDFSIWQKRPEQVAEHERQLQYWTEQLADSSPAELLTDLPRPLVPTGKAGIVQLTIEGAVYERLRAFCRVHQTTSFAVLLAAFRATHYRLTGAEDATIGSPIANRNRPELESLIGFFVNTQCIRVTIREDDTFDKLVQQVRATTTAAQVNQDVPFERIVSALMPGSRDTSRNPLVQLSFALHSQHDLGRIDLQDLTGEALPTPVFTRLDVEFHLFQQAEKFGGSVLFATDLFEPETIQGLVSVFQEVLRRGLEQPQTPIAVLPLDNASEDLRSMGLLQMERTNYPRDSSVVDVFRDQVAANPRAIAVKDSVLELTYAQLDEKSDQLAAWLCQHNIPAETIVGVLAPRSCETIIAFLGILKANLAYLPLDDNVPAARIETILSAVPGHTLVLLGSHVAAPSIGLADAEFVNINHTLGHSLQLNSTCAKLQPSATSLAYVIFTSGSTGKPKGVMIEHRSIVRLVKNSNTLAKLPRAARVAHQFNLAFDAANYEIYGTLLNGGALICVDYSTLLDIDALVAMFKREKITASSLSPGLLKQCVNSAPEMLKALQVIYTGGDRLDGRDAIELQALVPGGVYNMYGPTENTVISTLYNLGDKHSYVNGVPIGTTVSNSGAYVMDALQQLVPVGVMGELVVTGDGLARGYTDPELDRNRFIKVNIDGQVVRAYRTGDRVRYRRIDGQLEFFGRMDQQIKIRGFRIETAEVENAMLSHSAVRNAAVVVPTQDIQEKGMIGFVVIENNTPKNEESKEEHLLQTELAILNRMKSILPPYMLPSRIIILDQMPSNFNGKVDRKELDRMAQSVPRQKTTAGRIVPRNELEASLCKEFAEVLGVEVGITDNFFDLGGHSLLATKLAARISRRLDTRVSVKDVFDQPVPADLALKVSSYISQGHAMDNGTLSTTNSIPFQLLHFEDSQKFIDRDIVPQLAHQSAKIVDVYPVTWIQKHFLVDPATGLPRTPSLFFVDFPANADCDKICNASRSLIQLFDIFRTVFVQAAGNFYQVVLEELDIPISVIETEDISTATRVLKEQDQQNPLQFGQGFLRFAVVKTRSAVRLVLRISHCLYDGLSFEHVVQSLHALYNGDRIPTQPKFVQYVQHLTDSRKEGYDFWLSVLEESSMTVVETGRRAQQLSSPEGAWFVEKIIKAVIPANSDGITQATVFTTASTILLARMTGSSDITFSRLVSGRQSLPINDQHIVGPCTNIVPVRIRMTDGTNARELLGMVQDQYIDSLPFETLGFDDIKENCTKWPASTTNYGCCSTFQNFEMQPQSQVQDERVRLAGLTNFKDAELLNGATATNKRVLDDVPMHEIDMIGIPEPDGLHVRVVLTASRQIFEEEVVDRMHEEFCDIILGLNKILQK

SEQ ID NO: 38 - DNA, 1197 bp, Curvularia clavata
  CDS (1)..(1197)
atgacctttgtcgagactgtagccgtcccggacaatgaggagcgtccttcggctggacacaatcgtcctgtagccgacagcaccaagtgtcccaacgcgagggagatgaaggttcagaatcgtgtcgcccaaaggacacatcatcgccgtttaaaaacaaagctggaagtgctacgggaaagattgaaagagcctgagaagcaagttggggaacctgccagggtccagacatccacctccacgctggtgtcggatgcggcaaccagcttggcagattcgatgtgcttggtgccagcagtgcaaaatgaccaggccatggcgtttgatttcctgatgacgccatcaccttctgttggtaatgattgtccttcaaatgacctggaaaccatgcgccaagctgcgtctgttcattccaacaccttaggcggggccttcccgctaaacaggtcgccctgtactgagaacatgacgcccgaatcgcaagttagtttatctaccgcaccattatgttttacttctgtcgtcccggcggagttggacatggacgctttctgcacgcttgacagcagtgattggtcgcggccgaatgaagaatctctcctacgtttggccaattattctacctctgtgtcacctacaaacgttcaatggggcgtagatgagaatgctccgctccaagatcgtgtgcgctacatgagggaccaagccgtcgccatgggcttcggctctctcgatgacgtcgtcgaggcgcactacacacagaagcttgagtgcaccagcccatcgttccaagagcagcgactgagtcgcaatcggcgactgtcgcgactgttgagcacgctgcacaatgcagccaaagactggtcggagtgggagcgacgcgggttgcaagagcaagttacccaaggtgccgaagacatcttggtctccgagctaaattcgtacattacacagcgctcgatgaactcaacggacgacaaaatcatcacgggcggcctcctggacgagcagtctagactgaggcaggacgtggaagaaaggcggagactccaggacagtctccccaacctaggtgccctcctcaccactctgctgtcaaggtccaacgcacccaaccaagacgcccgtcgagacactgtactcgccatgatcaagacaatgtgctttgatcaagacgagaacatgagtatatcatag

SEQ ID NO: 39 - protein, 398 aa, Curvularia clavata
MTFVETVAVPDNEERPSAGHNRPVADSTKCPNAREMKVQNRVAQRTHHRRLKTKLEVLRERLKEPEKQVGEPARVQTSTSTLVSDAATSLADSMCLVPAVQNDQAMAFDFLMTPSPSVGNDCPSNDLETMRQAASVHSNTLGGAFPLNRSPCTENMTPESQVSLSTAPLCFTSVVPAELDMDAFCTLDSSDWSRPNEESLLRLANYSTSVSPTNVQWGVDENAPLQDRVRYMRDQAVAMGFGSLDDVVEAHYTQKLECTSPSFQEQRLSRNRRLSRLLSTLHNAAKDWSEWERRGLQEQVTQGAEDILVSELNSYITQRSMNSTDDKIITGGLLDEQSRLRQDVEERRRLQDSLPNLGALLTTLLSRSNAPNQDARRDTVLAMIKTMCFDQDENMSIS

SEQ ID NO: 40 - DNA, 1269 bp, Curvularia clavata
  CDS (1)..(1269)
atggacccgagacagtcacggatcacggagctggcaatagccatcaaaaagcagacggaaacactgcagtcactattggacagtctcaaagttgcgacgccttctttttctgtaaacgccaatcaggagttgcctcgcaatgcagctgttcagctcgcgcagtcctctatcctcgactcctgtacggaactgcaggatttggtcgaaggccctctggcacatgttgggcgaataatgagccctcgagttcatatatcgtcagctctgcaagctattgtacatttcaatatagcagagaaaatcgcaaaacacgagactatctcatttggcgagatcgcaaaaagatgcaaaatggacgtagatgatgtcaagcgaattatgcgattagccatctcgtaccgaatcttcaaagagtctcatatcggatttgtaaatcacacggctagctcattcttgattgcggaaaaccttcttgtgaggcaatggattagtctttgctgtgatgagttcataccagcgggttcgttccttgttcctgccatgaaaaaatggcctagctctgaagagcctaacgagaccgcgtttgcgctgcttcataagggagatagtctatgggaagtccttaaaaagcagcctgaaaaagctcagcgctttgctcacggaatggagtacatgcggacactcccgccattcgacatcaaccatctgtttacctcgttgaactgggagatcgactgtgagatggttttggtggacgtgggcggttctcaaggctccattgctgaagctttacttcgaagacacccgcgactacgatgttacgttcaagaccttccagagaccttgagcaaagccgtcgtgcccaaggatctcaagggtcgtcttgagttcgtaagccacagcatgttcaaagagcagcctataaaagccgacgtatacttgctcaggtcaattttgcacgactggttagatggatacgccctgcaaatcatccggaacctgattcccgctctcgaggttggatccaaggtgattataaatgagatctgtctaccggagccaaacgccatctcagcatatgaggcacagcttattcgcgggtacgatctttcaatgaagcaacaatttaattcgaaagagcgagatgtgcacgagtgggaaactctgttccgacttgcagacagacggttcaaactaaatcgcatcgtcaatccaccaggctcattccttgccgttctagaattcgaatggcaacccaccacaccataa

SEQ ID NO: 41 - protein, 422 aa, Curvularia clavata
MDPRQSRITELAIAIKKQTETLQSLLDSLKVATPSFSVNANQELPRNAAVQLAQSSILDSCTELQDLVEGPLAHVGRIMSPRVHISSALQAIVHFNIAEKIAKHETISFGEIAKRCKMDVDDVKRIMRLAISYRIFKESHIGFVNHTASSFLIAENLLVRQWISLCCDEFIPAGSFLVPAMKKWPSSEEPNETAFALLHKGDSLWEVLKKQPEKAQRFAHGMEYMRTLPPFDINHLFTSLNWEIDCEMVLVDVGGSQGSIAEALLRRHPRLRCYVQDLPETLSKAVVPKDLKGRLEFVSHSMFKEQPIKADVYLLRSILHDWLDGYALQIIRNLIPALEVGSKVIINEICLPEPNAISAYEAQLIRGYDLSMKQQFNSKERDVHEWETLFRLADRRFKLNRIVNPPGSFLAVLEFEWQPTTP

SEQ ID NO: 42 - DNA, 1617 bp, Curvularia clavata
  CDS (1)..(1617)
atgactgaacccacatggaagacagttgcatcggagaaacagcagcagcgtgaatccaaaatcccttcagaatggcaaattccgaagtcgtcgcatccagctcccgaagtaacctttgttcaagacttcccagccaaatcgggaatgttcaccaatcgagagctgcaactaacagcggcgactgcatcggatgtaacggccaagatctccactggcgaatggacggccgtggaggtcacgactgctgtgtgcaagcgagctgccgtggctcaacaattgttgaattgtgtaacggagatctgctttgatcaagctatagcaagagcgaaggagcttgacgcgtattttgaaaaagaaggaaagaccgtgggcccactccacggattaccaattagcttcaaagaccagttcaatgtcaaaggcttcgactccaccatcggctactgcagttatgctagcaagccagcaacggcagactcaactctcgtcaagctcctggtcaaggctggggcaatcatctatgtcaagtccaatgttcctatcacgctaatgatgggcgagtcattcaacaacatctttggacgcacactcaacccccgcaatcgggagttgaccacaggaggctcatcaggcggagaagcagcactggtcacgttctgtgccagcttcctcggtgtgggcaccgacatcggtggcagccttcgcataccatgctcattcaccgggctgtatgggctaagaccatcccacggcagagtgtcatatcaacatgtgcagaacaccttgctcggacaggaagcagtcagatcatgtgctggacccatgtgccgtgcaccggaagatatccgcttgttcatgtcgagtctagctgcccagcagccctggctttgggatccccagagtctgccactcccatggcgggcggaggaagaggtcttaccgaagaagttgtgtttcggttttgctctaggtgatggccatgtaggcccgaaaaagttaaagcaagcagggcatgctgtcattaacttcaatctcacagaaggaaaagaagtaaatgagatcatgaacaagatgttcactgcggatgggggtgccgagtttcagcgcgacaccgatgccacgggcgagcccctgccacctacagtagaatactggctcggccacagctcgcaaatcaaagcctcaaccgtaagcgagacatggaaaaatcagcacaagaaggcgttgcttgcgcaaaagttcctagagaagtggcaagcaaccaaagggcgaacgggcacgagtcgccctatcgatgggctgatcatgccatcgacgccatttccggccagtcgtcacggcagcggctggccatggcactttggtgatctctctgccctactagatctgaccacgggcgttttcccagtcacccgggtcaatctggagaaagacgccgtgccgccgagctggacgcccatgtctgtgaaagacaaggaggcgatggattactatgagaagccagagaatcacgagaatgccctagtcggcctccaattgattggtagaaggttggaggaggaaaaggtaacagctatgcttacgcttattaggaatgtgcttgaagtagattattaa

SEQ ID NO: 43 - protein, 538 aa, Curvularia clavata
MTEPTWKTVASEKQQQRESKIPSEWQIPKSSHPAPEVTFVQDFPAKSGMFTNRELQLTAATASDVTAKISTGEWTAVEVTTAVCKRAAVAQQLLNCVTEICFDQAIARAKELDAYFEKEGKTVGPLHGLPISFKDQFNVKGFDSTIGYCSYASKPATADSTLVKLLVKAGAIIYVKSNVPITLMMGESFNNIFGRTLNPRNRELTTGGSSGGEAALVTFCASFLGVGTDIGGSLRIPCSFTGLYGLRPSHGRVSYQHVQNTLLGQEAVRSCAGPMCRAPEDIRLFMSSLAAQQPWLWDPQSLPLPWRAEEEVLPKKLCFGFALGDGHVGPKKLKQAGHAVINFNLTEGKEVNEIMNKMFTADGGAEFQRDTDATGEPLPPTVEYWLGHSSQIKASTVSETWKNQHKKALLAQKFLEKWQATKGRTGTSRPIDGLIMPSTPFPASRHGSGWPWHFGDLSALLDLTTGVFPVTRVNLEKDAVPPSWTPMSVKDKEAMDYYEKPENHENALVGLQLIGRRLEEEKVTAMLTLIRNVLEVDY

SEQ ID NO: 44 - DNA, 2991 bp, Curvularia clavata
  CDS (1)..(2991)
atggcgttgcaagagcgccgtgccgcggtcacaagttccgatatcctctcagcgcatgctatctcgtctcccgccttggccgcagcggccatcaatttcgccgccagcttccatcgagatgcccgcacctgttgcagcgctcatgagcgtagccagctccagaaagtctaccgcgacaagatcctcgccaacgacaagtttacggccaacattgctgctgccttcctctctgtcctgggccccaacgccggccgtaacgatgcaggtgccgagcgcgagcgctggggcgactttgaccgcctggcgcagcgaggcaagaacatgcgcgaccgcgagagccagcatttgcaacatcagtcaggcatcattgccgcctgggggcctcgatgcttcgagtactacggctggcatgtcctgccgctgccgctgctgcgtcaggtgcacgaccttgccgtgctgatacctagctgggacgacgccgttgagctgctgaattccaggatgctgttgcgccacgaactgcgtgtgctgcacggcaacaacaaggccctccgaatcggtgaacactctgccgcttccaaagttcaggactcacgctcacctgttgagcgtaccgacatcgtggctgctctcgactgggctcgtgccaacgcaacttcggctgcggcacgtcaagcggtcaaggaagcggcgcagggcatgaatgggactccgatcaacacattcggtttgaagcgagattgctatggtatggtcgtaccgtcggtcggcccctacgatcctgatggagatgatgacaatgatgaagacgttgtcgatgtgtcccctcggccagcgaagcacatcaaattgtcagccgcagagccgcttcgtctgatgtttccaggttcattgagtcatgtccaggcttgtcaaagacatgacactgacggcgagaaggccagtactgcacccattcgtagtaacaaactgtcccagtccaaacagccagagctagacacagcagccgagagtcttcgtacgaggcatattcacaatgaacgcatcaacgagcccctcgacgaagtctcggactgcagtctatctctccaaacaatagccgtgggaggagggagcgctcaggaggaaacgccagaccaagatgtggaacatgcacatcctgaagttgagataacatccgccataagcagtgagcttaggaaggtagacgagcgtaccgatggtataaggatagggcgtgtgattatgaggcgcagtcactgtatggtaagagaacaggacaaccagactaacgaggaggggacaggagaagtacagtcacagcgggacaggagagcgagggacttgggaaaggatatggagacggatatggatattgacagccagctggaggagatgctggacatacatgctctggaggcgcaaagaaatcacgaagaaatgtcggatggtgaagatgttgttgcaggagtggcgggcccgggaacgccaacgcacagggcggcggaagaaggaggatgcagagaaaaagaagcagagaatgccaaaacggatgaggagcaagtgcaggacaaagcagctctggatcaggcgggaaatactaatacgaatcgagaggtagaaaacgcagcaccaaaagcgcacagccaagaaggtgccctgcgtgcatcgcgaacgggcacgatcgtggaaaggacagtggagttacactcaacgcactcaattcatcaaagagcgagtgtgaatacgacggctccaaccgtggcgcgatcaagcgatagcgacgacagcgattcactccattcacccacggcgcttcaaaatctgcaagcctatatcgataccagaactcaccaactcactcaagtgctgagccagctcaactcaacacctgacgtcagacaccacgctcaactgcagcttgactggttaagtccgcaacgatgggccagtgtctacgtggagccagaacatcacatgggcgccacttcctcagcatcatcagacagcgctgacatttggtgtctggactgggatacgttccaccagtatgctgacagcaaccatgtcttccggcggcctgttgttatcaagcaaaagttccaggacagcggtatgtatgaggttgacagatacgtggatatgctgtggcagcgctttccggagcagcatattgaggtccaaaacagcattacaggcactagtcgattgatgagcatggccgagtattgctctacggctttgactgttacggaggctggcacgagtctgtctgacaatactacctccgtgagcaacgctgttaaccttcgctgtctggctcgcgcagacgagccgctcttgacacggctcgagcgctttcaactgctctcgacgctcgcatctcgcgttgcaggcacaattggcaggaccgaacattctccacctagcaatctcgagagtctcctcggattcgacgcgctcagctttgccgacgcgttttcaagctcacatgccaatctctttggcggaagttgggtgcggtgcctcgatggcctcaagatttatgccatcgctgcagacttagatgcagaagactggcggcgcttcgcagatgaaggatacaaatggtcgcctcgaggcaaagggcgcttgatcgccctagaggaagacgatgttctgttcattccgcctggcctgcgggccatacatgccagcttcacgccagagccctgtttgatggaaggcggtatgctgtgggacgaatgcgccatccctgagatcttagacgagctgctctggattgcacgacaccaggcaggcactgtccagcctctcgaatttcagctttcaagtctgattgatgcgctggagcagtggttgaatgagaataaccacattaaccagtcgtcgccatcacacactgcagctgaagagcgtcagacgctcaaggctagcattcagtcgcttcgcgactgtttaagcggcagatcagcggctttcccatcttga

SEQ ID NO: 45 - protein, 996 aa, Curvularia clavata
MALQERRAAVTSSDILSAHAISSPALAAAAINFAASFHRDARTCCSAHERSQLQKVYRDKILANDKFTANIAAAFLSVLGPNAGRNDAGAERERWGDFDRLAQRGKNMRDRESQHLQHQSGIIAAWGPRCFEYYGWHVLPLPLLRQVHDLAVLIPSWDDAVELLNSRMLLRHELRVLHGNNKALRIGEHSAASKVQDSRSPVERTDIVAALDWARANATSAAARQAVKEAAQGMNGTPINTFGLKRDCYGMVVPSVGPYDPDGDDDNDEDVVDVSPRPAKHIKLSAAEPLRLMFPGSLSHVQACQRHDTDGEKASTAPIRSNKLSQSKQPELDTAAESLRTRHIHNERINEPLDEVSDCSLSLQTIAVGGGSAQEETPDQDVEHAHPEVEITSAISSELRKVDERTDGIRIGRVIMRRSHCMVREQDNQTNEEGTGEVQSQRDRRARDLGKDMETDMDIDSQLEEMLDIHALEAQRNHEEMSDGEDVVAGVAGPGTPTHRAAEEGGCREKEAENAKTDEEQVQDKAALDQAGNTNTNREVENAAPKAHSQEGALRASRTGTIVERTVELHSTHSIHQRASVNTTAPTVARSSDSDDSDSLHSPTALQNLQAYIDTRTHQLTQVLSQLNSTPDVRHHAQLQLDWLSPQRWASVYVEPEHHMGATSSASSDSADIWCLDWDTFHQYADSNHVFRRPVVIKQKFQDSGMYEVDRYVDMLWQRFPEQHIEVQNSITGTSRLMSMAEYCSTALTVTEAGTSLSDNTTSVSNAVNLRCLARADEPLLTRLERFQLLSTLASRVAGTIGRTEHSPPSNLESLLGFDALSFADAFSSSHANLFGGSWVRCLDGLKIYAIAADLDAEDWRRFADEGYKWSPRGKGRLIALEEDDVLFIPPGLRAIHASFTPEPCLMEGGMLWDECAIPEILDELLWIARHQAGTVQPLEFQLSSLIDALEQWLNENNHINQSSPSHTAAEERQTLKASIQSLRDCLSGRSAAFPS

SEQ ID NO: 46 - DNA, 234 bp, Curvularia clavata
  CDS (1)..(234)
atgtcaaacaagaagaacgagggccttgagaagggaggcaatgggtcggctgagcacgagagctttctgcccaagtcggcgcttcactaccgcgctcgcgtcgatggcggcacaagcggccttcttgcgcggctcgacaatagtcccggcgctgctgtcttggcttattgcttctcctcggtcagcacccttggatatgttccggactgcgaggataacctttgcggctcctaa

SEQ ID NO: 47 - protein, 77 aa, Curvularia clavata
MSNKKNEGLEKGGNGSAEHESFLPKSALHYRARVDGGTSGLLARLDNSPGAAVLAYCFSSVSTLGYVPDCEDNLCGS

SEQ ID NO: 48 - DNA, 4017 bp, Curvularia clavata
  CDS (1)..(4017)
atgagtgctatcgagctgccgccgctgcgctcgcggtctgaagaagcagcgagggcagaacacaatgcgcagacactcgcacacgaaaatgcaaatatcgcgggctatgatgagagcccggcagtccaacaagtcgagaccgatgctccagagactaaaggagccccgcaggcttctttcaagaattactttcgtgtcttttcatatgggacaaagcttgactactttttaatttcgctatgttgctttacgtctattggagcaggtactgcgatgccgctgatgaacattgtctttggcaagctcgtaggaaattttacagactacttcatcccaggatcaaatgtcacccgacaagaattcgaggcagagattaacaaactagccctctatatcttctacctcttcataggcaagtttgccatgtcgtacatttccatgctcgcaattcgaatcagcggtatgagaatatcggctgcgcttcgcctggcatacctgcgtgcactcttcgcccagccagtgagcgttatcgacaccgtcagtcccggcaaggttgccaatcgcatcacgacgtcatcgaatatcgtccagcttgctatctcgcagcattttgcaaccctgtttcagtctcttgccttcaccgtcggattatacgtggtggcgttagtaaaagggtggaagttgacgctgatcgcctcgacgggtctccctttcatcctaatcgtatacggcgccatgttcccgccctttctccggatccaccagatcaccgacaagttccaagaggaagcatcggctatggcgtatgaaatgttctcctccattaggatgattgtcgcctttggcaccgagtcgagacttgctaagcagcacggagtcatgctctccaaagctgcaagcaatgagaaaagagctgcgccgttaatgggcttgaccatgtctccggctatggtggccatgtacggtatcttcggtatcaccttctggttcggaatcaaggaatatacaaaagggagaatctcaagcgtcggcgacatcaccgttgtgctcttctcagtcatgatggccgtaatgaatattgggcgagtcgcgtctccgattatatccatcgcaaaagccgcgactgctgcgaccgagctctttgtcacaatcgacgcttcgttccacgatacatctggtgtcatggagcccgaggttacaggtaatgctgctatcactttcatcaatgttgctttttcgtaccccagccggccgggtgtcccaattctcaagggacttgatttgacaattactgctggcaaagtcactgccattgtaggtccatcggggtccgggaaaagcacgattgttggccttatccaacgatggtacgaccttctcggcacaacagctactgctaagaaaatcgacgagacagagattccttcatcatccactatggcgtccagcccaatagaagcagtctatgacaatacagacaagaaatccaaaaaggggaaggccggggaagaagaagaaccagaacaagatctcgggccaaatacgtgcactggctcgttgagtgttggtagaacaaatcttcgtaatgtggatgtaaggtggtggcgttcgcaaatcggcatggtccagcaggagcctttcctgttcaatgatacaatatacaacaatattgtgtttggactctgcgggacccgttatgaaggactgtccaaagatgaaaagaaaataatggtcgatgaggcgtgtcgcgaggcttgcgcggaggagtttatctcgcggctcccacaagggttggacacgcttgtgggcgagagcggcatcaaactttctggtggccagcgtcagcgtatcgccattgccaggagtattatcaaacgaccgcctattctcattctagacgaggcaacgagtgccatcgatgtcagaacggagcgaattgttcaagaagcgcttgatcgtgtttctaagaaccgtaccacgattgtcatcgcacatcgcctatccacaatcaaacgggcggacagcatagtcgtcttacggcagggccagctggttgagcaaggcacgcatgaagagctgctgaaaaacggagatggggtctattacggcttagttcatgcccaagagctggaaatggacgctgaagacgatgatgaccacagctcaagcttagagaacatcaaaatgaacgacactaaggaggacactgctagtagcggattcgagggacacgcttctagagaagattcaacatatcagaatgtaggtctacttcacagtctcggtcgacttgttgtagagcaacgtcaccattggatcctctacagcgtttgctgcataggcatactcggagccggcgcagtctacccactccaagcgtacattttcgcaaggattatcaacgtcttcacacttacaggtcccgagctcgtcaaacaaggcaacttctgggcaggcatgttcggcgtacttgcgggtggggttggactgtcgtactatctgcttggtgctgcctcacatctaatttctgtcgaattaacacgcaagtatcgatcagaatacctcagcaacatgatccgaaaaccaatcctcttttttgacgataaagttcacagcccaggctctcttacgtcaagactgagctcggacagtcaacaggtccagcagttgttgtcgatggagatgagcatggcgctcattgcctgcaccaaccttctcggatgtacaattatcgccttcgtttacggctggaagctttcccttgttggtttatttgctgccttgcctctcattcttggtgccggactcgtgcgcacgcgtctcgagatacaactcgaggctgagaacgcaaaagttttcgagaacagcagccagtttgccacagaagcggtggcaggtttccgcactgtgctaagtctgctcatggagccgatgattagaagccgctacgacaagttgctcaagggccacgttgtggaagctttggccaaggcaaaatatggtaccatcattttcgctgcaagtgacagtcttgagcttgcatgtatgtctctgaccttctggtacggcggaaaactccttgcgtctcgtgaatatgatctcattcagttcttcattgtctacacggccatcattcaaggcgctacggcagcaggaatctggttctcttttactccaagcatggctcaagcgacaggtgctgcaaaccgaatccttagcatgcggccgacatcgacggatccatcatcttactcgcctcttccatgctcagatgagggagtgggcattgaatttcaacacgtctccttcaaataccagtctcgagacgtgcccgttctttccaacctcaatctgcaaatcctaccgggtcaggttgctgcgttagtaggcagtagtggctgtggtaaatcaacaacactgtctcttctcgaacgcttctacgatgcgagttcgggccatattctatacaacgggcaagacatcaccacgttcagcccggcagagtaccggaaacaaatgagcctggtgagccaagagcccacgctctaccaaggcagcattcgagaaaacatatctctgagtgtagagtctgcatccgacgacgacatcaaacaggcctgccgtgatgcgcaaattcatgacttcatcacctcgcttccagaaggctacgagacgcgcttgggaccgaaaggaatgtctctctcaggtggtcaaagacagcgaatctctcttgccagggcgctgttgcgcaaaccaaaaatcctactcctcgatgaagcaaccagctcgctagattcagagagcgagaaatacgtccaggaagctatcgagcgagctgcaagcgagggtgacagaaccgtcataattgttgcgcataggctggctacaattcagaaggcggatgttatctttgtactgggcagtggaaaggtgctagagaagggggatcatcaggcactgctccggaaaaagggcgtgtactggcagatgtgtcaagcccaggccctcaatcgctga

SEQ ID NO: 49 - protein, 1338 aa, Curvularia clavata
MSAIELPPLRSRSEEAARAEHNAQTLAHENANIAGYDESPAVQQVETDAPETKGAPQASFKNYFRVFSYGTKLDYFLISLCCFTSIGAGTAMPLMNIVFGKLVGNFTDYFIPGSNVTRQEFEAEINKLALYIFYLFIGKFAMSYISMLAIRISGMRISAALRLAYLRALFAQPVSVIDTVSPGKVANRITTSSNIVQLAISQHFATLFQSLAFTVGLYVVALVKGWKLTLIASTGLPFILIVYGAMFPPFLRIHQITDKFQEEASAMAYEMFSSIRMIVAFGTESRLAKQHGVMLSKAASNEKRAAPLMGLTMSPAMVAMYGIFGITFWFGIKEYTKGRISSVGDITVVLFSVMMAVMNIGRVASPIISIAKAATAATELFVTIDASFHDTSGVMEPEVTGNAAITFINVAFSYPSRPGVPILKGLDLTITAGKVTAIVGPSGSGKSTIVGLIQRWYDLLGTTATAKKIDETEIPSSSTMASSPIEAVYDNTDKKSKKGKAGEEEEPEQDLGPNTCTGSLSVGRTNLRNVDVRWWRSQIGMVQQEPFLFNDTIYNNIVFGLCGTRYEGLSKDEKKIMVDEACREACAEEFISRLPQGLDTLVGESGIKLSGGQRQRIAIARSIIKRPPILILDEATSAIDVRTERIVQEALDRVSKNRTTIVIAHRLSTIKRADSIVVLRQGQLVEQGTHEELLKNGDGVYYGLVHAQELEMDAEDDDDHSSSLENIKMNDTKEDTASSGFEGHASREDSTYQNVGLLHSLGRLVVEQRHHWILYSVCCIGILGAGAVYPLQAYIFARIINVFTLTGPELVKQGNFWAGMFGVLAGGVGLSYYLLGAASHLISVELTRKYRSEYLSNMIRKPILFFDDKVHSPGSLTSRLSSDSQQVQQLLSMEMSMALIACTNLLGCTIIAFVYGWKLSLVGLFAALPLILGAGLVRTRLEIQLEAENAKVFENSSQFATEAVAGFRTVLSLLMEPMIRSRYDKLLKGHVVEALAKAKYGTIIFAASDSLELACMSLTFWYGGKLLASREYDLIQFFIVYTAIIQGATAAGIWFSFTPSMAQATGAANRILSMRPTSTDPSSYSPLPCSDEGVGIEFQHVSFKYQSRDVPVLSNLNLQILPGQVAALVGSSGCGKSTTLSLLERFYDASSGHILYNGQDITTFSPAEYRKQMSLVSQEPTLYQGSIRENISLSVESASDDDIKQACRDAQIHDFITSLPEGYETRLGPKGMSLSGGQRQRISLARALLRKPKILLLDEATSSLDSESEKYVQEAIERAASEGDRTVIIVAHRLATIQKADVIFVLGSGKVLEKGDHQALLRKKGVYWQMCQAQALNR

SEQ ID NO: 50 - DNA, 1047 bp, Curvularia clavata
  CDS (1)..(1047)
atgaagctcaccgttttcagtgcaaaaccctacgatatcgaatacctgggtggcatcgctactaatcaaaactcctcgcctgcaattgagatcaacttcctgcatgtcccgctctccagcgagacggccgcgttcgcgaacggcgctgatgccgtctgcgtcttcgttcacgatgtgcttgacgccaacgtcctccgcgaactatacgccgccggcgtgcgcgccattctcttccgctgctcagggtataacaatattgacctaagggaggctgagcgcttaggcttcttcgtcgccaacgtcccttcgtactcgccggaggcagtcgccgagttcgcagtcgcgctcatccaaacacttaaccggaagacgcaccgggcatacaaccgcgtgcgggacggcaatttcaacctcgacggcctactcggacgaacactacacggcaaaacagtcggcattgtagggtcaggccggatcggactcgccatggcgcagatcgttcagggcttcggatgcaagctgttggcatacgatcctcggcctacagaagccttcaagaagtacggcgaatacgtggatctcgatacgctgctgtcacaatgcgacattgtaagcttacactgcccgctgatggactcgacgcagcacatcatcaacgacacaactgtcagcaaaatgaagcgcggcgcgatgctcgtcaacacgtcgcgtggcgggctgatcgacacgcagagcgtgatgaaggcgctgaagagcaagcgtctgggcgggctagccctcgacgtttacgagggcgagcgcgcgctcttctacaaagaccattcgggtgacatcatccatgacgatttgctcatgcgcctcaccacgtttcacaacgtcgttgtgtctggccaccaggcgtatttcactgaagaggcactcacggaaattgcggagtgtacgctgaggaatctggatgattgggcgaagggagtgccaacggcgaatgcgctggtgcagggcaggaattcgaatgggaggagggagcgggggttggcgcggctctga

SEQ ID NO: 51 - protein, 348 aa, Curvularia clavata
MKLTVFSAKPYDIEYLGGIATNQNSSPAIEINFLHVPLSSETAAFANGADAVCVFVHDVLDANVLRELYAAGVRAILFRCSGYNNIDLREAERLGFFVANVPSYSPEAVAEFAVALIQTLNRKTHRAYNRVRDGNFNLDGLLGRTLHGKTVGIVGSGRIGLAMAQIVQGFGCKLLAYDPRPTEAFKKYGEYVDLDTLLSQCDIVSLHCPLMDSTQHIINDTTVSKMKRGAMLVNTSRGGLIDTQSVMKALKSKRLGGLALDVYEGERALFYKDHSGDIIHDDLLMRLTTFHNVVVSGHQAYFTEEALTEIAECTLRNLDDWAKGVPTANALVQGRNSNGRRERGLARL

SEQ ID NO: 52 - DNA, 936 bp, Curvularia clavata
  CDS (1)..(936)
atgacgaaaagggaaagcaacactctagcggttctcggatgcggtatggtttttcttgtatcattattagatctggctaacagactgttaggtgcgcttggcaccgccattctctcaggcatacttgcttctatggcagatcagacagccgatgattcgggtcgcctgtttacgaatttcactgcctgtgtgcgtcgcaaagagaccggtgctgctgttagtgataagatcagttcgcacgccaatgcaaacaaagtcgagatattgaacaaggaaaatctacggggcgtcaagcaagcagatgctgttctcttagcctgccaaacgcacctatacaaagctctgttcgacgagccagggatgcgagaggcactgaagaagaaactgatcatcagcgtgctggctggtgttaccacagcacaactcgaagcagcgctggggaatggtgaggattactttgtaatccgagctatgccaaatatcgcatgttttgtacgagattctgcaaccgtcatcgagaagcctcagcgaactttcccagaggcattgcttcacgtcaccgacaccgtcttcaaagccgtgggcaacgtcttttacatccaaccatctgcctatgacatatgtactgctctctgtggttcatcacccgcatttcttgcagtatttattgactctatggtggatggtgcggtagccatggggctaagtcacaaggacgcggtcgacatggcggcctgcacaatgaggggagctgccagtttggtgctagagagcggcaatccttggacgatacgacaccaggtggcgtcacctggaggctcgaccatgcagggtctactggcacttgaacaaggaaatgtgagatcaaccatctccaacgcgttgatggtcgccgcgaaagaagcaaaaaagctggggtcgaaagaaaacgcgtag

SEQ ID NO: 53 - protein, 311 aa, Curvularia clavata
MTKRESNTLAVLGCGMVFLVSLLDLANRLLGALGTAILSGILASMADQTADDSGRLFTNFTACVRRKETGAAVSDKISSHANANKVEILNKENLRGVKQADAVLLACQTHLYKALFDEPGMREALKKKLIISVLAGVTTAQLEAALGNGEDYFVIRAMPNIACFVRDSATVIEKPQRTFPEALLHVTDTVFKAVGNVFYIQPSAYDICTALCGSSPAFLAVFIDSMVDGAVAMGLSHKDAVDMAACTMRGAASLVLESGNPWTIRHQVASPGGSTMQGLLALEQGNVRSTISNALMVAAKEAKKLGSKENA

SEQ ID NO: 54 - DNA, 924 bp, Curvularia clavata
  CDS (1)..(924)
atggagagcgaagacaatccattgaggatacaaaccggctcgctctgctcattccaacgaccgactccgctggtactcattcacgactctagtggcacgacctttagttatttccgcctgggcagcttgaaccgtgatgtctgggctattcatgacccacactttgataaaagcacgccgtggaagggcgggtttggcgagattgccgagcactacataaaattgattgaaacggcaggaattcgaggttcgatcttgctcggaggatggtcgctcgggggttatctcgcgctcacgattgctcacaaattaacggctatcacaaatcctaccttctctgtcaccggcatcttgcttgttgactctccgtatcacaccccaatgagtaagctgccacctcacgccccagatcccaactttcaacaccttccggaactcgtccgtaagtcattcgagaattacgatgtccttttagacagatgggaactacctccatggaccgcgcctgctttggaaggcaaaactatacgttgtagcgcgggtggcaagaccttcacggtagcaaacggcaggatcctatacaagcccctaggtaagggctgggaagatgtcaaaatgcaaagcttcgagcatggcacctctactttggaacgctacatcgaattacccccagcagctctgatcagatgcgctcaggccataccaactgatacagattcgaaaatgccgtgtttcgtagatcgattccgtcacgagacactgctaggttgggatagtaatttccccagtttcatcaaggccgccgtggacacgaacactcaccacttcaacatattcgagtctcagaatctcaaacgattaacgatacaattgaatgaatgtctagaagttctagatagctgttgcccgatgggatactgctga

SEQ ID NO: 55 - protein, 307 aa, Curvularia clavata
MESEDNPLRIQTGSLCSFQRPTPLVLIHDSSGTTFSYFRLGSLNRDVWAIHDPHFDKSTPWKGGFGEIAEHYIKLIETAGIRGSILLGGWSLGGYLALTIAHKLTAITNPTFSVTGILLVDSPYHTPMSKLPPHAPDPNFQHLPELVRKSFENYDVLLDRWELPPWTAPALEGKTIRCSAGGKTFTVANGRILYKPLGKGWEDVKMQSFEHGTSTLERYIELPPAALIRCAQAIPTDTDSKMPCFVDRFRHETLLGWDSNFPSFIKAAVDTNTHHFNIFESQNLKRLTIQLNECLEVLDSCCPMGYC

SEQ ID NO: 56 - DNA, 33 bp, Artificial
  Synthetic DNA
cggtacccggggatctagtctgttgattactcg

SEQ ID NO: 57 - DNA, 35 bp, Artificial
  Synthetic DNA
ctcgacaaaggtcattttgactttgaataccggtg

SEQ ID NO: 58 - DNA, 22 bp, Artificial
  Synthetic DNA
gcagttgccgttggaccagagg

SEQ ID NO: 59 - DNA, 37 bp, Artificial
  Synthetic DNA
atagtcataacaagccgcgacactgtaatattaaagc

SEQ ID NO: 60 - DNA, 24 bp, Artificial
  Synthetic DNA
atgacctttgtcgagactgtagcc

SEQ ID NO: 61 - DNA, 39 bp, Artificial
  Synthetic DNA
tccaacggcaactgcctatgatatactcatgttctcgtc

SEQ ID NO: 62 - DNA, 35 bp, Artificial
  Synthetic DNA
cgactctagaggatcctgatggtcagatggatctg

SEQ ID NO: 63 - DNA, 28 bp, Artificial
  Synthetic DNA
gcttgttatgactatgtatacatatgcg

SEQ ID NO: 64 - DNA, 21 bp, Artificial
  Synthetic DNA
gacagactcttcgtcgacgtc

SEQ ID NO: 65 - DNA, 22 bp, Artificial
  Synthetic DNA
gttgtggttggtgttcctgagg

SEQ ID NO: 66 - DNA, 22 bp, Artificial
  Synthetic DNA
cactcgatctaccaaatcgacg

SEQ ID NO: 67 - DNA, 21 bp, Artificial
  Synthetic DNA
cctatccggatatgcagtcac

SEQ ID NO: 68 - DNA, 38 bp, Artificial
  Synthetic DNA
cggtacccggggatcctctgaagcggtcaaggataacg

SEQ ID NO: 69 - DNA, 37 bp, Artificial
  Synthetic DNA
atgaagcagagcggcgagcctaagatatgccaggagg

SEQ ID NO: 70 - DNA, 37 bp, Artificial
  Synthetic DNA
ctagcaaccgtcatgccatagacgtggcactcgaacg

SEQ ID NO: 71 - DNA, 38 bp, Artificial
  Synthetic DNA
cgactctagaggatccgtcttaaggatggttcagctgc

SEQ ID NO: 72 - DNA, 20 bp, Artificial
  Synthetic DNA
catgacggttgctagggtcg

SEQ ID NO: 73 - DNA, 20 bp, Artificial
  Synthetic DNA
gccgctctgcttcattgctg

SEQ ID NO: 74 - DNA, 33 bp, Artificial
  Synthetic DNA
cggtacccggggatcgacccattgcagcttgtg

SEQ ID NO: 75 - DNA, 37 bp, Artificial
  Synthetic DNA
atgaagcagagcggcgtgcagtatggtgtctaaaacg

SEQ ID NO: 76 - DNA, 36 bp, Artificial
  Synthetic DNA
ctagcaaccgtcatggatgaatgagcaccctgttag

SEQ ID NO: 77 - DNA, 39 bp, Artificial
  Synthetic DNA
cgactctagaggatcgtacattacaaaaacctgttgcag

SEQ ID NO: 78 - DNA, 35 bp, Artificial
  Synthetic DNA
cggtacccggggatcgtcccacgtgcagcttcaac

SEQ ID NO: 79 - DNA, 35 bp, Artificial
  Synthetic DNA
atgaagcagagcggccgtggagtatcccaggatgg

SEQ ID NO: 80 - DNA, 35 bp, Artificial
  Synthetic DNA
ctagcaaccgtcatgccagccaaagggtatcatgg

SEQ ID NO: 81 - DNA, 33 bp, Artificial
  Synthetic DNA
cgactctagaggatctgagggcagcgtagcctg

SEQ ID NO: 82 - DNA, 37 bp, Artificial
  Synthetic DNA
cggtacccggggatcgtggataaattcgtaccctttg

SEQ ID NO: 83 - DNA, 36 bp, Artificial
  Synthetic DNA
atgaagcagagcggcctgatctttgttgtggtcgtg

SEQ ID NO: 84 - DNA, 35 bp, Artificial
  Synthetic DNA
ctagcaaccgtcatgcagtttggcacttgagcatc

SEQ ID NO: 85 - DNA, 36 bp, Artificial
  Synthetic DNA
cgactctagaggatccacggaaaggaactcctacag

SEQ ID NO: 86 - DNA, 34 bp, Artificial
  Synthetic DNA
cggtacccggggatcctctgggaaaagcggttag

SEQ ID NO: 87 - DNA, 34 bp, Artificial
  Synthetic DNA
atgaagcagagcggcgaagaaccgagagcgagag

SEQ ID NO: 88 - DNA, 40 bp, Artificial
  Synthetic DNA
ctagcaaccgtcatgcttgcatctacctagatatttcacg

SEQ ID NO: 89 - DNA, 36 bp, Artificial
  Synthetic DNA
cgactctagaggatccagagaatcagcagagacacc

SEQ ID NO: 90 - DNA, 39 bp, Artificial
  Synthetic DNA
cggtacccggggatcccctggtagttcagtggaagtaag

SEQ ID NO: 91 - DNA, 34 bp, Artificial
  Synthetic DNA
atgaagcagagcggctgatagaggtacgggggtg

SEQ ID NO: 92 - DNA, 34 bp, Artificial
  Synthetic DNA
ctagcaaccgtcatgtgcttggctgcttcaaatc

SEQ ID NO: 93 - DNA, 39 bp, Artificial
  Synthetic DNA
cgactctagaggatcctaatacttgtcgtcccactgatg

SEQ ID NO: 94 - DNA, 34 bp, Artificial
  Synthetic DNA
cggtacccggggatcgcagtacatcgtcagggtc

SEQ ID NO: 95 - DNA, 36 bp, Artificial
  Synthetic DNA
atgaagcagagcggcgatgaataaggcgaaggaaag

SEQ ID NO: 96 - DNA, 37 bp, Artificial
  Synthetic DNA
ctagcaaccgtcatgccctcttttttcttgctgtctc

SEQ ID NO: 97 - DNA, 35 bp, Artificial
  Synthetic DNA
cgactctagaggatcgaaggaaggacggatactgg

SEQ ID NO: 98 - DNA, 39 bp, Artificial
  Synthetic DNA
cggtacccggggatcgatgagcgtagaattcgtaaaaag

SEQ ID NO: 99 - DNA, 32 bp, Artificial
  Synthetic DNA
atgaagcagagcggcgcgaacgggcgtttttc

SEQ ID NO: 100 - DNA, 35 bp, Artificial
  Synthetic DNA
ctagcaaccgtcatggaaggaaggacggatactgg

SEQ ID NO: 101 - DNA, 37 bp, Artificial
  Synthetic DNA
cgactctagaggatcccctcttttttcttgctgtctc

SEQ ID NO: 102 - DNA, 40 bp, Artificial
  Synthetic DNA
cggtacccggggatcctccttattttgcaacttctgatac

SEQ ID NO: 103 - DNA, 37 bp, Artificial
  Synthetic DNA
atgaagcagagcggccgtgttgattttggtaattttg

SEQ ID NO: 104 - DNA, 39 bp, Artificial
  Synthetic DNA
ctagcaaccgtcatggatgagcgtagaattcgtaaaaag

SEQ ID NO: 105 - DNA, 32 bp, Artificial
  Synthetic DNA
cgactctagaggatcgcgaacgggcgtttttc

SEQ ID NO: 106 - DNA, 37 bp, Artificial
  Synthetic DNA
cggtacccggggatccgtgttgattttggtaattttg

SEQ ID NO: 107 - DNA, 40 bp, Artificial
  Synthetic DNA
atgaagcagagcggcctccttattttgcaacttctgatac

SEQ ID NO: 108 - DNA, 39 bp, Artificial
  Synthetic DNA
ctagcaaccgtcatgctagcagccataagagacgtaacc

SEQ ID NO: 109 - DNA, 34 bp, Artificial
  Synthetic DNA
cgactctagaggatcgttttcattgcatgctccg

SEQ ID NO: 110 - DNA, 59 bp, Artificial
  Synthetic DNA
tcgacaagcttgcggccgccacgtgactagtatggccagcgacatcaatactcatccag

SEQ ID NO: 111 - DNA, 47 bp, Artificial
  Synthetic DNA
actagtcacgtggcggccgcggcgcgccaagatcgtcttgctgtacg

SEQ ID NO: 112 - DNA, 41 bp, Artificial
  Synthetic DNA
gatgcgctagcggccgcgaagtggtccttgtcgctggtgac

SEQ ID NO: 113 - DNA, 28 bp, Artificial
  Synthetic DNA
tgccgttcgcattcataggcatctcgtc

SEQ ID NO: 114 - DNA, 25 bp, Artificial
  Synthetic DNA
tgaatgcgaacggcaaggttgacag

SEQ ID NO: 115 - DNA, 25 bp, Artificial
  Synthetic DNA
cttggttgctggcttcgtcgttgtc

SEQ ID NO: 116 - DNA, 25 bp, Artificial
  Synthetic DNA
aagccagcaaccaagtcgaagattg

SEQ ID NO: 117 - DNA, 43 bp, Artificial
  Synthetic DNA
gtcactagtgcggccgcctatttttgcaagatcttgttcaaac

SEQ ID NO: 118 - DNA, 29 bp, Artificial
  Synthetic DNA
ggactagtatgactgaacccacatggaag

SEQ ID NO: 119 - DNA, 29 bp, Artificial
  Synthetic DNA
ggactagtttaataatctacttcaagcac

SEQ ID NO: 120 - DNA, 33 bp, Artificial
  Synthetic DNA
ataagaatgcggccgcatggcgttgcaagagcg

SEQ ID NO: 121 - DNA, 36 bp, Artificial
  Synthetic DNA
ataagaatgcggccgctcaagatgggaaagccgctg

SEQ ID NO: 122 - DNA, 28 bp, Artificial
  Synthetic DNA
ctagctagcatgagtgctatcgagctgc

SEQ ID NO: 123 - DNA, 28 bp, Artificial
  Synthetic DNA
ctagctagctcagcgattgagggcctgg

SEQ ID NO: 124 - DNA, 36 bp, Artificial
  Synthetic DNA
ataagaatgcggccgcatgaagctcaccgttttcag

SEQ ID NO: 125 - DNA, 32 bp, Artificial
  Synthetic DNA
ataagaatgcggccgctcagagccgcgccaac

SEQ ID NO: 126 - DNA, 29 bp, Artificial
  Synthetic DNA
ggactagtatgacgaaaagggaaagcaac

SEQ ID NO: 127 - DNA, 27 bp, Artificial
  Synthetic DNA
ggactagtctacgcgttttctttcgac

SEQ ID NO: 128 - DNA, 29 bp, Artificial
  Synthetic DNA
ctagctagcatggagagcgaagacaatcc

SEQ ID NO: 129 - DNA, 27 bp, Artificial
  Synthetic DNA
ctagctagctcagcagtatcccatcgg

SEQ ID NO: 130 - DNA, 36 bp, Artificial
  Synthetic DNA
atttgcggccgcatggacccgagacagtcacggatc

SEQ ID NO: 131 - DNA, 36 bp, Artificial
  Synthetic DNA
atttgcggccgcttatggtgtggtgggttgccattc

SEQ ID NO: 132 - DNA, 20 bp, Artificial
  Synthetic DNA
gacgccacgaacgcatagac

SEQ ID NO: 133 - DNA, 21 bp, Artificial
  Synthetic DNA
ttcccagagaggtagatcgac

SEQ ID NO: 134 - DNA, 20 bp, Artificial
  Synthetic DNA
gaccgttacagcgagttcag

SEQ ID NO: 135 - DNA, 20 bp, Artificial
  Synthetic DNA
ctgaattcctcgcacagaac

SEQ ID NO: 136 - DNA, 20 bp, Artificial
  Synthetic DNA
gaagttgagaacgccatgct

SEQ ID NO: 137 - DNA, 20 bp, Artificial
  Synthetic DNA
gatgcgagatgggagcatgt

SEQ ID NO: 138 - DNA, 20 bp, Artificial
  Synthetic DNA
gccctactagatctgaccac

SEQ ID NO: 139 - DNA, 20 bp, Artificial
  Synthetic DNA
gctgttaccttttcctcctc

SEQ ID NO: 140 - DNA, 20 bp, Artificial
  Synthetic DNA
agatcttagacgagctgctc

SEQ ID NO: 141 - DNA, 20 bp, Artificial
  Synthetic DNA
aaacagtcgcgaagcgactg

SEQ ID NO: 142 - DNA, 20 bp, Artificial
  Synthetic DNA
acgtccaggaagctatcgag

SEQ ID NO: 143 - DNA, 20 bp, Artificial
  Synthetic DNA
attgagggcctgggcttgac

SEQ ID NO: 144 - DNA, 20 bp, Artificial
  Synthetic DNA
gtgatgaaggcgctgaagag

SEQ ID NO: 145 - DNA, 20 bp, Artificial
  Synthetic DNA
ctccgcaatttccgtgagtg

SEQ ID NO: 146 - DNA, 20 bp, Artificial
  Synthetic DNA
tgactctatggtggatggtg

SEQ ID NO: 147 - DNA, 20 bp, Artificial
  Synthetic DNA
ccttgttcaagtgccagtag

SEQ ID NO: 148 - DNA, 20 bp, Artificial
  Synthetic DNA
gattccgtcacgagacactg

SEQ ID NO: 149 - DNA, 20 bp, Artificial
  Synthetic DNA
agtatcccatcgggcaacag

SEQ ID NO: 150 - DNA, 18 bp, Artificial
  Synthetic DNA
acgttcaagaccttccag

SEQ ID NO: 151 - DNA, 18 bp, Artificial
  Synthetic DNA
gttccggatgatttgcag